European Patent Application EP 4 389 226 A2, published June 26, 2024. Title: Bispecific Binding Molecules That Are Capable of Binding CD137 and Tumor Antigens, and Uses Thereof. Applicant: MacroGenics, Inc. The sequence listing filed with the application follows.

SEQUENCE LISTING (232 sequences)

SEQ ID NO: 1 - protein, 107 aa, Homo sapiens [sequence omitted]

SEQ ID NO: 2 - protein, 104 aa, Homo sapiens
  REGION 1..104: note = MISC_FEATURE - Human IgG CL Lambda Domain
QPKAAPSVTLFPPSSEELQANKATLVCLISDFYPGAVTVAWKADSSPVKAGVETTPSKQSNNKYAASSYLSLTPEQWKSHRSYSCQVTHEGSTVEKTVAPTECS

SEQ ID NO: 3 - protein, 98 aa, Homo sapiens
  REGION 1..98: note = MISC_FEATURE - Human IgG1 CH1 Domain
ASTKGPSVFPLAPSSKSTSGGTAALGCLVKDYFPEPVTVSWNSGALTSGVHTFPAVLQSSGLYSLSSVVTVPSSSLGTQTYICNVNHKPSNTKVDKRV

SEQ ID NO: 4 - protein, 98 aa, Homo sapiens
  REGION 1..98: note = MISC_FEATURE - Human IgG2 CH1 Domain
ASTKGPSVFPLAPCSRSTSESTAALGCLVKDYFPEPVTVSWNSGALTSGVHTFPAVLQSSGLYSLSSVVTVPSSNFGTQTYTCNVDHKPSNTKVDKTV

SEQ ID NO: 5 - protein, 98 aa, Homo sapiens
  REGION 1..98: note = MISC_FEATURE - Human IgG3 CH1 Domain
ASTKGPSVFPLAPCSRSTSGGTAALGCLVKDYFPEPVTVSWNSGALTSGVHTFPAVLQSSGLYSLSSVVTVPSSSLGTQTYTCNVNHKPSNTKVDKRV

SEQ ID NO: 6 - protein, 98 aa, Homo sapiens
  REGION 1..98: note = MISC_FEATURE - Human IgG4 CH1 Domain
ASTKGPSVFPLAPCSRSTSESTAALGCLVKDYFPEPVTVSWNSGALTSGVHTFPAVLQSSGLYSLSSVVTVPSSSLGTKTYTCNVDHKPSNTKVDKRV

SEQ ID NO: 7 - protein, 15 aa, Homo sapiens
  REGION 1..15: note = MISC_FEATURE - Human IgG1 Hinge Region
EPKSCDKTHTCPPCP

SEQ ID NO: 8 - protein, 12 aa, Homo sapiens
  REGION 1..12: note = MISC_FEATURE - Human IgG2 Hinge Region
ERKCCVECPPCP

SEQ ID NO: 9 - protein, 62 aa, Homo sapiens
  REGION 1..62: note = MISC_FEATURE - Human IgG3 Hinge Region
ELKTPLGDTTHTCPRCPEPKSCDTPPPCPRCPEPKSCDTPPPCPRCPEPKSCDTPPPCPRCP

SEQ ID NO: 10 - protein, 12 aa, Homo sapiens
  REGION 1..12: note = MISC_FEATURE - Human IgG4 Hinge Region
ESKYGPPCPSCP

SEQ ID NO: 11 - protein, 12 aa, synthetic construct
  REGION 1..12: note = Human IgG4 Hinge Region Variant Comprising S228P Substitution
ESKYGPPCPPCP

SEQ ID NO: 12 - protein, 217 aa, Homo sapiens
  REGION 1..217: note = MISC_FEATURE - Exemplary Human IgG1 CH2-CH3 Domain
  SITE 217: note = MISC_FEATURE - Xaa is Lysine (K) or Is Absent
APELLGGPSVFLFPPKPKDTLMISRTPEVTCVVVDVSHEDPEVKFNWYVDGVEVHNAKTKPREEQYNSTYRVVSVLTVLHQDWLNGKEYKCKVSNKALPAPIEKTISKAKGQPREPQVYTLPPSREEMTKNQVSLTCLVKGFYPSDIAVEWESNGQPENNYKTTPPVLDSDGSFFLYSKLTVDKSRWQQGNVFSCSVMHEALHNHYTQKSLSLSPGX

SEQ ID NO: 13 - protein, 216 aa, Homo sapiens
  REGION 1..216: note = MISC_FEATURE - Exemplary Human IgG2 CH2-CH3 Domain
  SITE 216: note = MISC_FEATURE - Xaa is Lysine (K) or Is Absent
APPVAGPSVFLFPPKPKDTLMISRTPEVTCVVVDVSHEDPEVQFNWYVDGVEVHNAKTKPREEQFNSTFRVVSVLTVVHQDWLNGKEYKCKVSNKGLPAPIEKTISKTKGQPREPQVYTLPPSREEMTKNQVSLTCLVKGFYPSDISVEWESNGQPENNYKTTPPMLDSDGSFFLYSKLTVDKSRWQQGNVFSCSVMHEALHNHYTQKSLSLSPGX

SEQ ID NO: 14 - protein, 217 aa, Homo sapiens
  REGION 1..217: note = MISC_FEATURE - Exemplary Human IgG3 CH2-CH3 Domain
  SITE 217: note = MISC_FEATURE - Xaa is Lysine (K) or Is Absent
APELLGGPSVFLFPPKPKDTLMISRTPEVTCVVVDVSHEDPEVQFKWYVDGVEVHNAKTKPREEQYNSTFRVVSVLTVLHQDWLNGKEYKCKVSNKALPAPIEKTISKTKGQPREPQVYTLPPSREEMTKNQVSLTCLVKGFYPSDIAVEWESSGQPENNYNTTPPMLDSDGSFFLYSKLTVDKSRWQQGNIFSCSVMHEALHNRFTQKSLSLSPGX

SEQ ID NO: 15 - protein, 217 aa, Homo sapiens
  REGION 1..217: note = MISC_FEATURE - Exemplary Human IgG1 CH2-CH3 Domain
  SITE 217: note = MISC_FEATURE - Xaa is Lysine (K) or Is Absent
APEFLGGPSVFLFPPKPKDTLMISRTPEVTCVVVDVSQEDPEVQFNWYVDGVEVHNAKTKPREEQFNSTYRVVSVLTVLHQDWLNGKEYKCKVSNKGLPSSIEKTISKAKGQPREPQVYTLPPSQEEMTKNQVSLTCLVKGFYPSDIAVEWESNGQPENNYKTTPPVLDSDGSFFLYSRLTVDKSRWQEGNVFSCSVMHEALHNHYTQKSLSLSLGX

SEQ ID NO: 16 - protein, 8 aa, synthetic construct
  REGION 1..8: note = Preferred Intervening Spacer Peptide (Linker 1)
GGGSGGGG

SEQ ID NO: 17 - protein, 15 aa, synthetic construct
  REGION 1..15: note = Intervening Spacer Peptide (Linker 1) for scFv Molecules
GGGGSGGGGSGGGGS

SEQ ID NO: 18 - protein, 6 aa, synthetic construct
  REGION 1..6: note = Preferred Intervening Spacer Peptide (Linker 2)
GGCGGG

SEQ ID NO: 19 - protein, 5 aa, synthetic construct
  REGION 1..5: note = Alternative Intervening Spacer Peptide (Linker 2)
ASTKG

SEQ ID NO: 20 - protein, 10 aa, synthetic construct
  REGION 1..10: note = Preferred Heterodimer-Promoting Domain (Linker 3)
DKTHTCPPCP

SEQ ID NO: 21 - protein, 13 aa, synthetic construct
  REGION 1..13: note = Alternative Heterodimer-Promoting Domain (Linker 3)
GGGDKTHTCPPCP

SEQ ID NO: 22 - protein, 5 aa, synthetic construct
  REGION 1..5: note = Preferred Intervening Spacer Peptide (Linker 4)
APSSS

SEQ ID NO: 23 - protein, 8 aa, synthetic construct
  REGION 1..8: note = Alternative Preferred Intervening Spacer Peptide (Linker 4)
APSSSPME

SEQ ID NO: 24 - protein, 11 aa, synthetic construct
  REGION 1..11: note = Alternative Preferred Intervening Spacer Peptide (Linker 4)
GGGSGGGSGGG

SEQ ID NO: 25 - protein, 6 aa, synthetic construct
  REGION 1..6: note = Alternative Linker
LGGGSG

SEQ ID NO: 26 - protein, 4 aa, synthetic construct
  REGION 1..4: note = Alternative Linker
GGGS

SEQ ID NO: 27 - protein, 6 aa, synthetic construct
  REGION 1..6: note = Alternative Linker
LEPKSS

SEQ ID NO: 28 - protein, 16 aa, synthetic construct
  REGION 1..16: note = Alternative Linker
VEPKSADKTHTCPPCP

SEQ ID NO: 29 - protein, 16 aa, synthetic construct
  REGION 1..16: note = Alternative Linker
LEPKSADKTHTCPPCP

SEQ ID NO: 30 - protein, 16 aa, synthetic construct
  REGION 1..16: note = Alternative Linker
LEPKSSDKTHTCPPCP

SEQ ID NO: 31 - protein, 7 aa, synthetic construct
  REGION 1..7: note = Preferred Heterodimer-Promoting Domain
GVEPKSC

SEQ ID NO: 32 - protein, 6 aa, synthetic construct
  REGION 1..6: note = Preferred Heterodimer-Promoting Domain
VEPKSC

SEQ ID NO: 33 - protein, 6 aa, synthetic construct
  REGION 1..6: note = Preferred Heterodimer-Promoting Domain
AEPKSC

SEQ ID NO: 34 - protein, 7 aa, synthetic construct
  REGION 1..7: note = Preferred Heterodimer-Promoting Domain
GFNRGEC

SEQ ID NO: 35 - protein, 6 aa, synthetic construct
  REGION 1..6: note = Preferred Heterodimer-Promoting Domain
FNRGEC

SEQ ID NO: 36 - protein, 28 aa, synthetic construct
  REGION 1..28: note = E-Coil Heterodimer-Promoting Domain
EVAALEKEVAALEKEVAALEKEVAALEK

SEQ ID NO: 37 - protein, 28 aa, synthetic construct
  REGION 1..28: note = K-Coil Heterodimer-Promoting Domain
KVAALKEKVAALKEKVAALKEKVAALKE

SEQ ID NO: 38 - protein, 28 aa, synthetic construct
  REGION 1..28: note = Cysteine-Containing E-Coil Heterodimer-Promoting Domain
EVAACEKEVAALEKEVAALEKEVAALEK

SEQ ID NO: 39 - protein, 28 aa, synthetic construct
  REGION 1..28: note = Cysteine-Containing K-Coil Heterodimer-Promoting Domain
KVAACKEKVAALKEKVAALKEKVAALKE

SEQ ID NO: 40 - protein, 217 aa, synthetic construct
  REGION 1..217: note = Human IgG1 CH2-CH3 Domain Variant Comprising Kabat L234A and L235A Substitutions
  SITE 217: note = MISC_FEATURE - Xaa is Lysine (K) or Is Absent
APEAAGGPSVFLFPPKPKDTLMISRTPEVTCVVVDVSHEDPEVKFNWYVDGVEVHNAKTKPREEQYNSTYRVVSVLTVLHQDWLNGKEYKCKVSNKALPAPIEKTISKAKGQPREPQVYTLPPSREEMTKNQVSLTCLVKGFYPSDIAVEWESNGQPENNYKTTPPVLDSDGSFFLYSKLTVDKSRWQQGNVFSCSVMHEALHNHYTQKSLSLSPGX

SEQ ID NO: 41 - protein, 217 aa, synthetic construct
  REGION 1..217: note = Human IgG1 CH2-CH3 Domain Variant Comprising Kabat M252Y, S254T and T256E Substitutions
  SITE 217: note = MISC_FEATURE - Xaa is Lysine (K) or Is Absent
APELLGGPSVFLFPPKPKDTLYITREPEVTCVVVDVSHEDPEVKFNWYVDGVEVHNAKTKPREEQYNSTYRVVSVLTVLHQDWLNGKEYKCKVSNKALPAPIEKTISKAKGQPREPQVYTLPPSREEMTKNQVSLTCLVKGFYPSDIAVEWESNGQPENNYKTTPPVLDSDGSFFLYSKLTVDKSRWQQGNVFSCSVMHEALHNHYTQKSLSLSPGX

SEQ ID NO: 42 - protein, 217 aa, synthetic construct
  REGION 1..217: note = Human IgG1 CH2-CH3 Domain Variant Comprising Kabat L234A, L235A, M252Y, S254T and T256E Substitutions
  SITE 217: note = MISC_FEATURE - Xaa is Lysine (K) or Is Absent
APEAAGGPSVFLFPPKPKDTLYITREPEVTCVVVDVSHEDPEVKFNWYVDGVEVHNAKTKPREEQYNSTYRVVSVLTVLHQDWLNGKEYKCKVSNKALPAPIEKTISKAKGQPREPQVYTLPPSREEMTKNQVSLTCLVKGFYPSDIAVEWESNGQPENNYKTTPPVLDSDGSFFLYSKLTVDKSRWQQGNVFSCSVMHEALHNHYTQKSLSLSPGX

SEQ ID NO: 43 - protein, 217 aa, synthetic construct
  REGION 1..217: note = Human IgG4 CH2-CH3 Domain Variant Comprising Kabat M252Y, S254T and T256E Substitutions
  SITE 217: note = misc_feature - Xaa can be any naturally occurring amino acid
APEFLGGPSVFLFPPKPKDTLYITREPEVTCVVVDVSQEDPEVQFNWYVDGVEVHNAKTKPREEQFNSTYRVVSVLTVLHQDWLNGKEYKCKVSNKGLPSSIEKTISKAKGQPREPQVYTLPPSQEEMTKNQVSLTCLVKGFYPSDIAVEWESNGQPENNYKTTPPVLDSDGSFFLYSRLTVDKSRWQEGNVFSCSVMHEALHNHYTQKSLSLSLGX

SEQ ID NO: 44 - protein, 217 aa, synthetic construct
  REGION 1..217: note = Exemplary "Knob-Bearing" IgG1 CH2-CH3 Domain
  SITE 217: note = MISC_FEATURE - Xaa is Lysine (K) or Is Absent
APEAAGGPSVFLFPPKPKDTLMISRTPEVTCVVVDVSHEDPEVKFNWYVDGVEVHNAKTKPREEQYNSTYRVVSVLTVLHQDWLNGKEYKCKVSNKALPAPIEKTISKAKGQPREPQVYTLPPSREEMTKNQVSLWCLVKGFYPSDIAVEWESNGQPENNYKTTPPVLDSDGSFFLYSKLTVDKSRWQQGNVFSCSVMHEALHNHYTQKSLSLSPGX

SEQ ID NO: 45 - protein, 217 aa, synthetic construct
  REGION 1..217: note = Exemplary "Knob-Bearing" IgG1 CH2-CH3 Domain
  SITE 217: note = MISC_FEATURE - Xaa is Lysine (K) or Is Absent
APEFLGGPSVFLFPPKPKDTLYITREPEVTCVVVDVSQEDPEVQFNWYVDGVEVHNAKTKPREEQFNSTYRVVSVLTVLHQDWLNGKEYKCKVSNKGLPSSIEKTISKAKGQPREPQVYTLPPSQEEMTKNQVSLWCLVKGFYPSDIAVEWESNGQPENNYKTTPPVLDSDGSFFLYSRLTVDKSRWQEGNVFSCSVMHEALHNHYTQKSLSLSLGX

SEQ ID NO: 46 - protein, 217 aa, synthetic construct
  REGION 1..217: note = Exemplary "Knob-Bearing" IgG1 CH2-CH3 Domain
  SITE 217: note = MISC_FEATURE - Xaa is Lysine (K) or Is Absent
APEAAGGPSVFLFPPKPKDTLYITREPEVTCVVVDVSHEDPEVKFNWYVDGVEVHNAKTKPREEQYNSTYRVVSVLTVLHQDWLNGKEYKCKVSNKALPAPIEKTISKAKGQPREPQVYTLPPSREEMTKNQVSLWCLVKGFYPSDIAVEWESNGQPENNYKTTPPVLDSDGSFFLYSKLTVDKSRWQQGNVFSCSVMHEALHNHYTQKSLSLSPGX

SEQ ID NO: 47 - protein, 217 aa, synthetic construct
  REGION 1..217: note = Exemplary "Hole-Bearing" IgG1 CH2-CH3 Domain
  SITE 217: note = MISC_FEATURE - Xaa is Lysine (K) or Is Absent
APEAAGGPSVFLFPPKPKDTLMISRTPEVTCVVVDVSHEDPEVKFNWYVDGVEVHNAKTKPREEQYNSTYRVVSVLTVLHQDWLNGKEYKCKVSNKALPAPIEKTISKAKGQPREPQVYTLPPSREEMTKNQVSLSCAVKGFYPSDIAVEWESNGQPENNYKTTPPVLDSDGSFFLVSKLTVDKSRWQQGNVFSCSVMHEALHNRYTQKSLSLSPGX

SEQ ID NO: 48 - protein, 217 aa, synthetic construct
  REGION 1..217: note = Exemplary "Hole-Bearing" IgG1 CH2-CH3 Domain
  SITE 217: note = MISC_FEATURE - Xaa is Lysine (K) or Is Absent
APEFLGGPSVFLFPPKPKDTLYITREPEVTCVVVDVSQEDPEVQFNWYVDGVEVHNAKTKPREEQFNSTYRVVSVLTVLHQDWLNGKEYKCKVSNKGLPSSIEKTISKAKGQPREPQVYTLPPSQEEMTKNQVSLSCAVKGFYPSDIAVEWESNGQPENNYKTTPPVLDSDGSFFLVSRLTVDKSRWQEGNVFSCSVMHEALHNRYTQKSLSLSLGX

SEQ ID NO: 49 - protein, 217 aa, synthetic construct
  REGION 1..217: note = Exemplary "Hole-Bearing" IgG1 CH2-CH3 Domain
  SITE 217: note = MISC_FEATURE - Xaa is Lysine (K) or Is Absent
APEAAGGPSVFLFPPKPKDTLYITREPEVTCVVVDVSHEDPEVKFNWYVDGVEVHNAKTKPREEQYNSTYRVVSVLTVLHQDWLNGKEYKCKVSNKALPAPIEKTISKAKGQPREPQVYTLPPSREEMTKNQVSLSCAVKGFYPSDIAVEWESNGQPENNYKTTPPVLDSDGSFFLVSKLTVDKSRWQQGNVFSCSVMHEALHNRYTQKSLSLSPGX

SEQ ID NO: 50 - protein, 46 aa, Streptococcus dysgalactiae
  REGION 1..46: note = MISC_FEATURE - Albumin-Binding Domain 3 (ABD3) of Protein G of Streptococcus Strain G148
LAEAKVLANRELDKYGVSDYYKNLIDNAKSAEGVKALIDEILAALP

SEQ ID NO: 51 - protein, 46 aa, synthetic construct; identical to SEQ ID NO: 50
  REGION 1..46: note = Deimmunized Albumin-Binding Domain 3 (ABD3) of Protein G of Streptococcus Strain G148

SEQ ID NO: 52 - protein, 46 aa, synthetic construct
  REGION 1..46: note = Deimmunized Albumin-Binding Domain 3 (ABD3) of Protein G of Streptococcus Strain G148
LAEAKVLANRELDKYGVSDYYKNAANNAKTVEGVKALIAEILAALP

SEQ ID NO: 53 - protein, 46 aa, synthetic construct
  REGION 1..46: note = Deimmunized Albumin-Binding Domain 3 (ABD3) of Protein G of Streptococcus Strain G148
LAEAKVLANRELDKYGVSDYYKNLISNAKSVEGVKALIAEILAALP

SEQ ID NO: 54 - protein, 120 aa, synthetic construct
  REGION 1..120: note = VH Domain of Margetuximab
QVQLQQSGPELVKPGASLKLSCTASGFNIKDTYIHWVKQRPEQGLEWIGRIYPTNGYTRYDPKFQDKATITADTSSNTAYLQVSRLTSEDTAVYYCSRWGGDGFYAMDYWGQGASVTVSS

SEQ ID NO: 55 - protein, 107 aa, synthetic construct
  REGION 1..107: note = VL Domain of Margetuximab
DIVMTQSHKFMSTSVGDRVSITCKASQDVNTAVAWYQQKPGHSPKLLIYSASFRYTGVPDRFTGSRSGTDFTFTISSVQAEDLAVYYCQQHYTTPPTFGGGTKVEIK

SEQ ID NO: 56 - protein, 120 aa, synthetic construct [sequence omitted]

SEQ ID NO: 57 - protein, 107 aa, synthetic construct [sequence omitted]

SEQ ID NO: 58 - protein, 119 aa, synthetic construct [sequence omitted]

SEQ ID NO: 59 - protein, 107 aa, synthetic construct [sequence omitted]

SEQ ID NO: 60 - protein, 119 aa, Mus musculus
  REGION 1..119: note = MISC_FEATURE - Murine Anti-HER2/neu Monoclonal Antibody HER2-MAB-1 VH Domain
EVQLQESGPELKKPGETVKISCKASGYTFTNYGMNWVKQAPGKGLKWMGWINTNIGEPTYTEEFKGRFAFSLGTSASTAFLQINNLKNEDTATYFCARDDGYGNRVSYWGQGTLVTVSA

SEQ ID NO: 61 - protein, 107 aa, Mus musculus
  REGION 1..107: note = MISC_FEATURE - Murine Anti-HER2/neu Monoclonal Antibody HER2-MAB-1 VL Domain
DILMTQSPLSMYTSLGERVTITCKASQDINSYLSWFQQKPGKSPKTLIYRANRLVDGVPSRFSGSGSGQDYSLTISSLEYEDMGIYYCLQHDEFPWTFGGGTKLEIK

SEQ ID NO: 62 - protein, 119 aa, synthetic construct
  REGION 1..119: note = Humanized Anti-HER2/neu Monoclonal Antibody hHER2-MAB-1 VH Domain
  SITE 100: note = MISC_FEATURE - Xaa is Asparatate (D) or Glutamate (E)
  SITE 101: note = MISC_FEATURE - Xaa is Glycine (G) or Isoleucine (I)
QVQLVQSGAEVKKPGASVKVSCKASGYTFTNYGMNWVRQAPGQGLEWMGWINTNIGEPTYTEEFKGRVTMTRDTSISTAYMELSRLRSDDTAVYYCARDXXYGNRVSYWGQGTLVTVSS

SEQ ID NO: 63 - protein, 107 aa, synthetic construct
  REGION 1..107: note = Humanized Anti-HER2/neu Monoclonal Antibody hHER2-MAB-1 VL Domain
  SITE 30: note = MISC_FEATURE - Xaa is Asparagine (N) or Serine (S)
  SITE 31: note = MISC_FEATURE - Xaa is Serine (S), Threonine (T) or Asparagine (N)
  SITE 55: note = MISC_FEATURE - Xaa is Valine (V) or Glutamine (Q)
  SITE 56: note = MISC_FEATURE - Xaa is Aspartate (D), Glutamate (E) or Serine (S)
DIQMTQSPSSLSASVGDRVTITCKASQDIXXYLSWFQQKPGKAPKTLIYRANRLXXGVPSRFSGSGSGTDFTLTISSLQPEDFATYYCLQHDEFPWTFGQGTKLEIK

SEQ ID NO: 64 - protein, 119 aa, synthetic construct
  REGION 1..119: note = Humanized Anti-HER2/neu Monoclonal Antibody hHER2-MAB-1 VH1 Domain
QVQLVQSGAEVKKPGASVKVSCKASGYTFTNYGMNWVRQAPGQGLEWMGWINTNIGEPTYTEEFKGRVTMTRDTSISTAYMELSRLRSDDTAVYYCARDDGYGNRVSYWGQGTLVTVSS

SEQ ID NO: 65 - protein, 119 aa, synthetic construct
  REGION 1..119: note = Humanized Anti-HER2/neu Monoclonal Antibody hHER2-MAB-1 VH2 Domain
QVQLVQSGAEVKKPGASVKVSCKASGYTFTNYGMNWVRQAPGQGLEWMGWINTNIGEPTYTEEFKGRVTMTRDTSISTAYMELSRLRSDDTAVYYCARDEGYGNRVSYWGQGTLVTVSS

SEQ ID NO: 66 - protein, 119 aa, synthetic construct
  REGION 1..119: note = Humanized Anti-HER2/neu Monoclonal Antibody hHER2-MAB-1 VH3 Domain
QVQLVQSGAEVKKPGASVKVSCKASGYTFTNYGMNWVRQAPGQGLEWMGWINTNIGEPTYTEEFKGRVTMTRDTSISTAYMELSRLRSDDTAVYYCARDDIYGNRVSYWGQGTLVTVSS

SEQ ID NO: 67 - protein, 107 aa, synthetic construct
  REGION 1..107: note = Humanized Anti-HER2/neu Monoclonal Antibody hHER2-MAB-1 VL1 Domain
DIQMTQSPSSLSASVGDRVTITCKASQDINSYLSWFQQKPGKAPKTLIYRANRLVDGVPSRFSGSGSGTDFTLTISSLQPEDFATYYCLQHDEFPWTFGQGTKLEIK

SEQ ID NO: 68 - protein, 107 aa, synthetic construct
  REGION 1..107: note = Humanized Anti-HER2/neu Monoclonal Antibody hHER2-MAB-1 VL2 Domain
DIQMTQSPSSLSASVGDRVTITCKASQDINTYLSWFQQKPGKAPKTLIYRANRLVEGVPSRFSGSGSGTDFTLTISSLQPEDFATYYCLQHDEFPWTFGQGTKLEIK

SEQ ID NO: 69 - protein, 107 aa, synthetic construct
  REGION 1..107: note = Humanized Anti-HER2/neu Monoclonal Antibody hHER2-MAB-1 VL3 Domain
DIQMTQSPSSLSASVGDRVTITCKASQDISNYLSWFQQKPGKAPKTLIYRANRLQSGVPSRFSGSGSGTDFTLTISSLQPEDFATYYCLQHDEFPWTFGQGTKLEIK

SEQ ID NO: 70 - protein, 121 aa, synthetic construct [sequence omitted]

SEQ ID NO: 71 - protein, 109 aa, synthetic construct [sequence omitted]

SEQ ID NO: 72 - protein, 116 aa, synthetic construct
  REGION 1..116: note = VH Domain of CD137 MAB-2 (CD137 MAB-2 VH)
EVQLVQSGAEVKKPGESLRISCKGSGYSFSTYWISWVRQMPGKGLEWMGKIYPGDSYTNYSPSFQGQVTISADKSISTAYLQWSSLKASDTAMYYCARGYGIFDYWGQGTLVTVSS

SEQ ID NO: 73 - protein, 108 aa, synthetic construct
  REGION 1..108: note = VL Domain of CD137 MAB-2 (CD137 MAB-2 VL)
SYELTQPPSVSVSPGQTASITCSGDNIGDQYAHWYQQKPGQSPVLVIYQDKNRPSGIPERFSGSNSGNTATLTISGTQAMDEADYYCATYTGFGSLAVFGGGTKLTVL

SEQ ID NO: 74 - protein, 119 aa, Mus musculus
  REGION 1..119: note = MISC_FEATURE - VH Domain of CD137 MAB-3 (CD137 MAB-3 VH)
QVQLQQPGAELVRPGASVKLSCKASGYTFTSYWINWVKQRPGQGLEWIGNIYPSDSYTNYNQKFKDKATLTVDKSSSTAYMQLSSPTSEDSAVYYCTRDYGSSYSFDYWGQGTTLTVSS

SEQ ID NO: 75 - protein, 107 aa, Mus musculus
  REGION 1..107: note = MISC_FEATURE - VL Domain of CD137 MAB-3 (CD137 MAB-3 VL)
DIQMTQTTSSLSASLGDRVTISCRPSQDISNYLNWYQQKPDGTVKLLIYYTSRLRSGVPSRFSGSGSGTDYSLTISNLEQEDIATYFCQQGDTLPYTFGGGTKLEIK

SEQ ID NO: 76 - protein, 119 aa, synthetic construct
  REGION 1..119: note = VH Domain of Humanized CD137 MAB-3 (hCD137 MAB-3 VH1)
QVQLVQSGAEVKKPGASVKVSCKASGYTFTSYWINWVKQAPGQGLEWIGNIYPSDSYTNYNQKFKDKATITADKSTSTAYMELSSLRSEDTAVYYCTRDYGSSYSFDYWGQGTTVTVSS

SEQ ID NO: 77 - protein, 119 aa, synthetic construct
  REGION 1..119: note = VH Domain of Optimized Humanized CD137 MAB-3 (hCD137 MAB-3 VH1)
  SITE 103: note = MISC_FEATURE - Xaa is Alanine (A) or Serine (S)
  SITE 104: note = MISC_FEATURE - Xaa is Tyrosine (Y)
  SITE 105: note = MISC_FEATURE - Xaa is Serine (S)
  SITE 106: note = MISC_FEATURE - Xaa is Phenylalanine (F), Methionine (M) or Tyrosine (Y)
  SITE 107: note = MISC_FEATURE - Xaa is Histidine (H), Serine (S) or Asparagine (N)
  SITE 108: note = MISC_FEATURE - Xaa is Proline (P), Threonine (T), Leucine or Valine (V)
QVQLVQSGAEVKKPGASVKVSCKASGYTFTSYWINWVKQAPGQGLEWIGNIYPSDSYTNYNQKFKDKATITADKSTSTAYMELSSLRSEDTAVYYCTRDYGSXXXXXXWGQGTTVTVSS

SEQ ID NO: 78 - protein, 6 aa, synthetic construct
  REGION 1..6: note = Preferred Residues 103-108 of SEQ ID NO:77 Variant 1A
AYSFHP

SEQ ID NO: 79 - protein, 6 aa, synthetic construct
  REGION 1..6: note = Preferred Residues 103-108 of SEQ ID NO:77 Variant 1B
AYSMST

SEQ ID NO: 80 - protein, 6 aa, synthetic construct
  REGION 1..6: note = Preferred Residues 103-108 of SEQ ID NO:77 Variant 1C
AYSYSL

SEQ ID NO: 81 - protein, 6 aa, synthetic construct
  REGION 1..6: note = Preferred Residues 103-108 of SEQ ID NO:77 Variant 1D
SYSYNV

SEQ ID NO: 82 - protein, 107 aa, synthetic construct
  REGION 1..107: note = VL Domain of Optimized Humanized Antibody hCD137 MAB-3 (hCD137 MAB-3 VL)
  SITE 41: note = MISC_FEATURE - Xaa is Asparatate (D) or Glycine (G)
  SITE 42: note = MISC_FEATURE - Xaa is Glycine (G) or Lysine (K)
DIQMTQSPSSLSASVGDRVTITCRPSQDISNYLNWYQQKPXXTVKLLIYYTSRLRSGVPSRFSGSGSGTDFTFTISSLQPEDIATYFCQQGDTLPYTFGQGTKLEIK

SEQ ID NO: 83 - protein, 119 aa, synthetic construct
  REGION 1..119: note = hCD137 MAB-3 VH1A
QVQLVQSGAEVKKPGASVKVSCKASGYTFTSYWINWVKQAPGQGLEWIGNIYPSDSYTNYNQKFKDKATITADKSTSTAYMELSSLRSEDTAVYYCTRDYGSAYSFHPWGQGTTVTVSS

SEQ ID NO: 84 - protein, 119 aa, synthetic construct
  REGION 1..119: note = hCD137 MAB-3 VH1B
QVQLVQSGAEVKKPGASVKVSCKASGYTFTSYWINWVKQAPGQGLEWIGNIYPSDSYTNYNQKFKDKATITADKSTSTAYMELSSLRSEDTAVYYCTRDYGSAYSMSTWGQGTTVTVSS

SEQ ID NO: 85 - protein, 119 aa, synthetic construct
  REGION 1..119: note = hCD137 MAB-3 VH1C
QVQLVQSGAEVKKPGASVKVSCKASGYTFTSYWINWVKQAPGQGLEWIGNIYPSDSYTNYNQKFKDKATITADKSTSTAYMELSSLRSEDTAVYYCTRDYGSAYSYSLWGQGTTVTVSS

SEQ ID NO: 86 - protein, 119 aa, synthetic construct
  REGION 1..119: note = hCD137 MAB-3 VH1D
QVQLVQSGAEVKKPGASVKVSCKASGYTFTSYWINWVKQAPGQGLEWIGNIYPSDSYTNYNQKFKDKATITADKSTSTAYMELSSLRSEDTAVYYCTRDYGSSYSYNVWGQGTTVTVSS

SEQ ID NO: 87 - protein, 107 aa, synthetic construct
  REGION 1..107: note = hCD137 MAB-3 VL1
DIQMTQSPSSLSASVGDRVTITCRPSQDISNYLNWYQQKPDGTVKLLIYYTSRLRSGVPSRFSGSGSGTDFTFTISSLQPEDIATYFCQQGDTLPYTFGQGTKLEIK

SEQ ID NO: 88 - protein, 107 aa, synthetic construct
  REGION 1..107: note = hCD137 MAB-3 VL2
DIQMTQSPSSLSASVGDRVTITCRPSQDISNYLNWYQQKPGGTVKLLIYYTSRLRSGVPSRFSGSGSGTDFTFTISSLQPEDIATYFCQQGDTLPYTFGQGTKLEIK

SEQ ID NO: 89 - protein, 107 aa, synthetic construct
  REGION 1..107: note = hCD137 MAB-3 VL3
DIQMTQSPSSLSASVGDRVTITCRPSQDISNYLNWYQQKPDKTVKLLIYYTSRLRSGVPSRFSGSGSGTDFTFTISSLQPEDIATYFCQQGDTLPYTFGQGTKLEIK

SEQ ID NO: 90 - protein, 123 aa, Mus musculus
  REGION 1..123: note = MISC_FEATURE - VH Domain of CD137 MAB-4 (CD137 MAB-4 VH)
QVQLQQPGAELVRPGASVKLSCKASGYTFTSYWINWVKQRPGQGLEWIGNIYPSDSYTNYDQKFKDKATLTVDKSSSTAYMQLSSPTSEDSAVYYCTKSGEYGKIGYYAMDYWGQGTSVTVSS

SEQ ID NO: 91 - protein, 107 aa, Mus musculus
  REGION 1..107: note = MISC_FEATURE - VL Domain of CD137 MAB-4 (CD137 MAB-4 VL)
DIQMTQTTSSLSASLGDRVTISCRASQDISNYLNWYQQKPDGTVKLLIYYTSRLHSGVPSRFSGSGSGTDYSLTISNLEQEDIATYFCQQGNTLPYTFGGGTKLEIK

SEQ ID NO: 92 - protein, 123 aa, synthetic construct
  REGION 1..123: note = VH Domain of Humanized CD137 MAB-4 (hCD137 MAB-4 VH1)
QVQLVQSGAEVKKPGASVKVSCKASGYTFTSYWINWVRQAPGQGLEWMGNIYPSDSYTNYDQKFKDRVTMTRDTSTSTVYMELSSLRSEDTAVYYCTKSGEYGKIGYYAMDYWGQGTTVTVSS

SEQ ID NO: 93 - protein, 107 aa, synthetic construct
  REGION 1..107: note = VL Domain of Humanized CD137 MAB-4 (hCD137 MAB-4 VL)
  SITE 87: note = MISC_FEATURE - Xaa is Phenylalanine (F) or Tyrosine (Y)
DIQMTQSPSSLSASVGDRVTITCRASQDISNYLNWYQQKPDKTVKLLIYYTSRLHSGVPSRFSGSGSGTDYTLTISSLQPEDIATYXCQQGNTLPYTFGQGTKLEIK

SEQ ID NO: 94 - protein, 107 aa, synthetic construct
  REGION 1..107: note = VL Domain of Humanized CD137 MAB-4 (hCD137 MAB-4 VL1)
DIQMTQSPSSLSASVGDRVTITCRASQDISNYLNWYQQKPDKTVKLLIYYTSRLHSGVPSRFSGSGSGTDYTLTISSLQPEDIATYFCQQGNTLPYTFGQGTKLEIK

SEQ ID NO: 95 - protein, 107 aa, synthetic construct
  REGION 1..107: note = VL Domain of Humanized CD137 MAB-4 (hCD137 MAB-4 VL2)
DIQMTQSPSSLSASVGDRVTITCRASQDISNYLNWYQQKPDKTVKLLIYYTSRLHSGVPSRFSGSGSGTDYTLTISSLQPEDIATYYCQQGNTLPYTFGQGTKLEIK

SEQ ID NO: 96 - protein, 111 aa, Mus musculus
  REGION 1..111: note = MISC_FEATURE - VH Domain of CD137 MAB-5 (CD137 MAB-5 VH)
QVQLKESGPGLVAPSQSLSITCTVSGFSLTSYDISWIRQPPGKGLEWLGVVWTGGGTNYNSAFMSRLSISKDNSKSQVFLKMNSLQTDDTAIYYCERVDYWGQGTSVTVSS

SEQ ID NO: 97 - protein, 112 aa, Mus musculus
  REGION 1..112: note = MISC_FEATURE - VL Domain of CD137 MAB-5 (CD137 MAB-5 VL)
DVVMTQTPLSLPVSLGDQASISCRSSQSLVHSNGNTYLHWYLQKPGQSPKLLIYKVSNRFSGVPDRFSGSGSGTDFTLKISRVEAEDLGVYFCSQSTHVPWTFGGGTKLEIK

SEQ ID NO: 98 - protein, 500 aa, synthetic construct
  REGION 1..500: note = First and Third Polypeptide Chains of DART-A
DIQMTQSPSSLSASVGDRVTITCKASQDINTYLSWFQQKPGKAPKTLIYRANRLVEGVPSRFSGSGSGTDFTLTISSLQPEDFATYYCLQHDEFPWTFGQGTKLEIKGGGSGGGGQVQLVQSGAEVKKPGASVKVSCKASGYTFTSYWINWVKQAPGQGLEWIGNIYPSDSYTNYNQKFKDKATITADKSTSTAYMELSSLRSEDTAVYYCTRDYGSSYSFDYWGQGTTVTVSSGGCGGGEVAACEKEVAALEKEVAALEKEVAALEKLEPKSADKTHTCPPCPAPEAAGGPSVFLFPPKPKDTLMISRTPEVTCVVVDVSHEDPEVKFNWYVDGVEVHNAKTKPREEQYNSTYRVVSVLTVLHQDWLNGKEYKCKVSNKALPAPIEKTISKAKGQPREPQVYTLPPSREEMTKNQVSLTCLVKGFYPSDIAVEWESNGQPENNYKTTPPVLDSDGSFFLYSKLTVDKSRWQQGNVFSCSVMHEALHNHYTQKSLSLSPG

SEQ ID NO: 99 - protein, 268 aa, synthetic construct
  REGION 1..268: note = Second and Fourth Polypeptide Chains of DART-A
DIQMTQSPSSLSASVGDRVTITCRPSQDISNYLNWYQQKPDGTVKLLIYYTSRLRSGVPSRFSGSGSGTDFTFTISSLQPEDIATYFCQQGDTLPYTFGQGTKLEIKGGGSGGGGQVQLVQSGAEVKKPGASVKVSCKASGYTFTNYGMNWVRQAPGQGLEWMGWINTNIGEPTYTEEFKGRVTMTRDTSISTAYMELSRLRSDDTAVYYCARDDGYGNRVSYWGQGTLVTVSSGGCGGGKVAACKEKVAALKEKVAALKEKVAALKE

SEQ ID NO: 100 - protein, 500 aa, synthetic construct
  REGION 1..500: note = First and Third Polypeptide Chain of DART-B
DIQMTQSPSSLSASVGDRVTITCKASQDISNYLSWFQQKPGKAPKTLIYRANRLQSGVPSRFSGSGSGTDFTLTISSLQPEDFATYYCLQHDEFPWTFGQGTKLEIKGGGSGGGGQVQLVQSGAEVKKPGASVKVSCKASGYTFTSYWINWVKQAPGQGLEWIGNIYPSDSYTNYNQKFKDKATITADKSTSTAYMELSSLRSEDTAVYYCTRDYGSSYSFDYWGQGTTVTVSSGGCGGGEVAACEKEVAALEKEVAALEKEVAALEKLEPKSADKTHTCPPCPAPEAAGGPSVFLFPPKPKDTLMISRTPEVTCVVVDVSHEDPEVKFNWYVDGVEVHNAKTKPREEQYNSTYRVVSVLTVLHQDWLNGKEYKCKVSNKALPAPIEKTISKAKGQPREPQVYTLPPSREEMTKNQVSLTCLVKGFYPSDIAVEWESNGQPENNYKTTPPVLDSDGSFFLYSKLTVDKSRWQQGNVFSCSVMHEALHNHYTQKSLSLSPG

SEQ ID NO: 101 - protein, 268 aa, synthetic construct
  REGION 1..268: note = Second and Fourth Polypeptide Chain of DART-B
DIQMTQSPSSLSASVGDRVTITCRPSQDISNYLNWYQQKPDKTVKLLIYYTSRLRSGVPSRFSGSGSGTDFTFTISSLQPEDIATYFCQQGDTLPYTFGQGTKLEIKGGGSGGGGQVQLVQSGAEVKKPGASVKVSCKASGYTFTNYGMNWVRQAPGQGLEWMGWINTNIGEPTYTEEFKGRVTMTRDTSISTAYMELSRLRSDDTAVYYCARDDGYGNRVSYWGQGTLVTVSSGGCGGGKVAACKEKVAALKEKVAALKEKVAALKE

SEQ ID NO: 102 - protein, 500 aa, synthetic construct
  REGION 1..500: note = First and Third Polypeptide Chains of DART-C
DIQMTQSPSSLSASVGDRVTITCRPSQDISNYLNWYQQKPDKTVKLLIYYTSRLRSGVPSRFSGSGSGTDFTFTISSLQPEDIATYFCQQGDTLPYTFGQGTKLEIKGGGSGGGGQVQLVQSGAEVKKPGASVKVSCKASGYTFTNYGMNWVRQAPGQGLEWMGWINTNIGEPTYTEEFKGRVTMTRDTSISTAYMELSRLRSDDTAVYYCARDDGYGNRVSYWGQGTLVTVSSGGCGGGEVAACEKEVAALEKEVAALEKEVAALEKLEPKSADKTHTCPPCPAPEAAGGPSVFLFPPKPKDTLMISRTPEVTCVVVDVSHEDPEVKFNWYVDGVEVHNAKTKPREEQYNSTYRVVSVLTVLHQDWLNGKEYKCKVSNKALPAPIEKTISKAKGQPREPQVYTLPPSREEMTKNQVSLTCLVKGFYPSDIAVEWESNGQPENNYKTTPPVLDSDGSFFLYSKLTVDKSRWQQGNVFSCSVMHEALHNHYTQKSLSLSPG

SEQ ID NO: 103 - protein, 268 aa, synthetic construct
  REGION 1..268: note = Second and Fourth Polypeptide Chains of DART-C
DIQMTQSPSSLSASVGDRVTITCKASQDISNYLSWFQQKPGKAPKTLIYRANRLQSGVPSRFSGSGSGTDFTLTISSLQPEDFATYYCLQHDEFPWTFGQGTKLEIKGGGSGGGGQVQLVQSGAEVKKPGASVKVSCKASGYTFTSYWINWVKQAPGQGLEWIGNIYPSDSYTNYNQKFKDKATITADKSTSTAYMELSSLRSEDTAVYYCTRDYGSSYSFDYWGQGTTVTVSSGGCGGGKVAACKEKVAALKEKVAALKEKVAALKE

SEQ ID NO: 104 - protein, 449 aa, synthetic construct
  REGION 1..449: note = First Polypeptide Chain of DART-D
QVQLVQSGAEVKKPGASVKVSCKASGYTFTNYGMNWVRQAPGQGLEWMGWINTNIGEPTYTEEFKGRVTMTRDTSISTAYMELSRLRSDDTAVYYCARDDGYGNRVSYWGQGTLVTVSSASTKGPSVFPLAPSSKSTSGGTAALGCLVKDYFPEPVTVSWNSGALTSGVHTFPAVLQSSGLYSLSSVVTVPSSSLGTQTYICNVNHKPSNTKVDKRVEPKSCDKTHTCPPCPAPEAAGGPSVFLFPPKPKDTLMISRTPEVTCVVVDVSHEDPEVKFNWYVDGVEVHNAKTKPREEQYNSTYRVVSVLTVLHQDWLNGKEYKCKVSNKALPAPIEKTISKAKGQPREPQVYTLPPSREEMTKNQVSLSCAVKGFYPSDIAVEWESNGQPENNYKTTPPVLDSDGSFFLVSKLTVDKSRWQQGNVFSCSVMHEALHNRYTQKSLSLSPGK

SEQ ID NO: 105 - protein, 214 aa, synthetic construct
  REGION 1..214: note = Second and Fifth Polypeptide Chains of DART-D
DIQMTQSPSSLSASVGDRVTITCKASQDISNYLSWFQQKPGKAPKTLIYRANRLQSGVPSRFSGSGSGTDFTLTISSLQPEDFATYYCLQHDEFPWTFGQGTKLEIKRTVAAPSVFIFPPSDEQLKSGTASVVCLLNNFYPREAKVQWKVDNALQSGNSQESVTEQDSKDSTYSLSSTLTLSKADYEKHKVYACEVTHQGLSSPVTKSFNRGEC

SEQ ID NO: 106 - protein, 727 aa, synthetic construct
  REGION 1..727: note = Third Polypeptide Chain of DART-D
QVQLVQSGAEVKKPGASVKVSCKASGYTFTNYGMNWVRQAPGQGLEWMGWINTNIGEPTYTEEFKGRVTMTRDTSISTAYMELSRLRSDDTAVYYCARDDGYGNRVSYWGQGTLVTVSSASTKGPSVFPLAPSSKSTSGGTAALGCLVKDYFPEPVTVSWNSGALTSGVHTFPAVLQSSGLYSLSSVVTVPSSSLGTQTYICNVNHKPSNTKVDKRVEPKSCDKTHTCPPCPAPEAAGGPSVFLFPPKPKDTLMISRTPEVTCVVVDVSHEDPEVKFNWYVDGVEVHNAKTKPREEQYNSTYRVVSVLTVLHQDWLNGKEYKCKVSNKALPAPIEKTISKAKGQPREPQVYTLPPSREEMTKNQVSLWCLVKGFYPSDIAVEWESNGQPENNYKTTPPVLDSDGSFFLYSKLTVDKSRWQQGNVFSCSVMHEALHNHYTQKSLSLSPGGGGSGGGSGGGDIQMTQTTSSLSASLGDRVTISCRPSQDISNYLNWYQQKPDGTVKLLIYYTSRLRSGVPSRFSGSGSGTDYSLTISNLEQEDIATYFCQQGDTLPYTFGGGTKLEIKGGGSGGGGQVQLQQPGAELVRPGASVKLSCKASGYTFTSYWINWVKQRPGQGLEWIGNIYPSDSYTNYNQKFKDKATLTVDKSSSTAYMQLSSPTSEDSAVYYCTRDYGSSYSFDYWGQGTTLTVSSGGCGGGEVAALEKEVAALEKEVAALEKEVAALEK

SEQ ID NO: 107 - protein, 268 aa, synthetic construct
  REGION 1..268: note = Fourth Polypeptide Chain of DART-D
DIQMTQTTSSLSASLGDRVTISCRPSQDISNYLNWYQQKPDGTVKLLIYYTSRLRSGVPSRFSGSGSGTDYSLTISNLEQEDIATYFCQQGDTLPYTFGGGTKLEIKGGGSGGGGQVQLQQPGAELVRPGASVKLSCKASGYTFTSYWINWVKQRPGQGLEWIGNIYPSDSYTNYNQKFKDKATLTVDKSSSTAYMQLSSPTSEDSAVYYCTRDYGSSYSFDYWGQGTTLTVSSGGCGGGKVAALKEKVAALKEKVAALKEKVAALKE

SEQ ID NO: 108 - protein, 449 aa, synthetic construct
  REGION 1..449: note = First Polypeptide Chain of DART-E
QVQLQQPGAELVRPGASVKLSCKASGYTFTSYWINWVKQRPGQGLEWIGNIYPSDSYTNYNQKFKDKATLTVDKSSSTAYMQLSSPTSEDSAVYYCTRDYGSSYSFDYWGQGTTLTVSSASTKGPSVFPLAPSSKSTSGGTAALGCLVKDYFPEPVTVSWNSGALTSGVHTFPAVLQSSGLYSLSSVVTVPSSSLGTQTYICNVNHKPSNTKVDKRVEPKSCDKTHTCPPCPAPEAAGGPSVFLFPPKPKDTLMISRTPEVTCVVVDVSHEDPEVKFNWYVDGVEVHNAKTKPREEQYNSTYRVVSVLTVLHQDWLNGKEYKCKVSNKALPAPIEKTISKAKGQPREPQVYTLPPSREEMTKNQVSLSCAVKGFYPSDIAVEWESNGQPENNYKTTPPVLDSDGSFFLVSKLTVDKSRWQQGNVFSCSVMHEALHNRYTQKSLSLSPGK

SEQ ID NO: 109 - protein, 214 aa, synthetic construct
  REGION 1..214: note = Second and Fifth Polypeptide Chain of DART-E
DIQMTQTTSSLSASLGDRVTISCRPSQDISNYLNWYQQKPDGTVKLLIYYTSRLRSGVPSRFSGSGSGTDYSLTISNLEQEDIATYFCQQGDTLPYTFGGGTKLEIKRTVAAPSVFIFPPSDEQLKSGTASVVCLLNNFYPREAKVQWKVDNALQSGNSQESVTEQDSKDSTYSLSSTLTLSKADYEKHKVYACEVTHQGLSSPVTKSFNRGEC

SEQ ID NO: 110 - protein, 727 aa, synthetic construct
  REGION 1..727: note = Third Polypeptide Chain of DART-E
QVQLQQPGAELVRPGASVKLSCKASGYTFTSYWINWVKQRPGQGLEWIGNIYPSDSYTNYNQKFKDKATLTVDKSSSTAYMQLSSPTSEDSAVYYCTRDYGSSYSFDYWGQGTTLTVSSASTKGPSVFPLAPSSKSTSGGTAALGCLVKDYFPEPVTVSWNSGALTSGVHTFPAVLQSSGLYSLSSVVTVPSSSLGTQTYICNVNHKPSNTKVDKRVEPKSCDKTHTCPPCPAPEAAGGPSVFLFPPKPKDTLMISRTPEVTCVVVDVSHEDPEVKFNWYVDGVEVHNAKTKPREEQYNSTYRVVSVLTVLHQDWLNGKEYKCKVSNKALPAPIEKTISKAKGQPREPQVYTLPPSREEMTKNQVSLWCLVKGFYPSDIAVEWESNGQPENNYKTTPPVLDSDGSFFLYSKLTVDKSRWQQGNVFSCSVMHEALHNHYTQKSLSLSPGGGGSGGGSGGGDIQMTQSPSSLSASVGDRVTITCKASQDISNYLSWFQQKPGKAPKTLIYRANRLQSGVPSRFSGSGSGTDFTLTISSLQPEDFATYYCLQHDEFPWTFGQGTKLEIKGGGSGGGGQVQLVQSGAEVKKPGASVKVSCKASGYTFTNYGMNWVRQAPGQGLEWMGWINTNIGEPTYTEEFKGRVTMTRDTSISTAYMELSRLRSDDTAVYYCARDDGYGNRVSYWGQGTLVTVSSGGCGGGEVAALEKEVAALEKEVAALEKEVAALEK

SEQ ID NO: 111 - protein, 268 aa, synthetic construct
  REGION 1..268: note = Fourth Polypeptide Chain of DART-E
DIQMTQSPSSLSASVGDRVTITCKASQDISNYLSWFQQKPGKAPKTLIYRANRLQSGVPSRFSGSGSGTDFTLTISSLQPEDFATYYCLQHDEFPWTFGQGTKLEIKGGGSGGGGQVQLVQSGAEVKKPGASVKVSCKASGYTFTNYGMNWVRQAPGQGLEWMGWINTNIGEPTYTEEFKGRVTMTRDTSISTAYMELSRLRSDDTAVYYCARDDGYGNRVSYWGQGTLVTVSSGGCGGGKVAALKEKVAALKEKVAALKEKVAALKE

SEQ ID NO: 112 - protein, 731 aa, synthetic construct
  REGION 1..731: note = Third Polypeptide Chain of DART-F
QVQLVQSGAEVKKPGASVKVSCKASGYTFTNYGMNWVRQAPGQGLEWMGWINTNIGEPTYTEEFKGRVTMTRDTSISTAYMELSRLRSDDTAVYYCARDDGYGNRVSYWGQGTLVTVSSASTKGPSVFPLAPSSKSTSGGTAALGCLVKDYFPEPVTVSWNSGALTSGVHTFPAVLQSSGLYSLSSVVTVPSSSLGTQTYICNVNHKPSNTKVDKRVEPKSCDKTHTCPPCPAPEAAGGPSVFLFPPKPKDTLMISRTPEVTCVVVDVSHEDPEVKFNWYVDGVEVHNAKTKPREEQYNSTYRVVSVLTVLHQDWLNGKEYKCKVSNKALPAPIEKTISKAKGQPREPQVYTLPPSREEMTKNQVSLWCLVKGFYPSDIAVEWESNGQPENNYKTTPPVLDSDGSFFLYSKLTVDKSRWQQGNVFSCSVMHEALHNHYTQKSLSLSPGGGGSGGGSGGGDIQMTQTTSSLSASLGDRVTISCRASQDISNYLNWYQQKPDGTVKLLIYYTSRLHSGVPSRFSGSGSGTDYSLTISNLEQEDIATYFCQQGNTLPYTFGGGTKLEIKGGGSGGGGQVQLQQPGAELVRPGASVKLSCKASGYTFTSYWINWVKQRPGQGLEWIGNIYPSDSYTNYDQKFKDKATLTVDKSSSTAYMQLSSPTSEDSAVYYCTKSGEYGKIGYYAMDYWGQGTSVTVSSGGCGGGEVAALEKEVAALEKEVAALEKEVAALEK

SEQ ID NO: 113 - protein, 272 aa, synthetic construct
  REGION 1..272: note = Fourth Polypeptide Chain of DART-F
DIQMTQTTSSLSASLGDRVTISCRASQDISNYLNWYQQKPDGTVKLLIYYTSRLHSGVPSRFSGSGSGTDYSLTISNLEQEDIATYFCQQGNTLPYTFGGGTKLEIKGGGSGGGGQVQLQQPGAELVRPGASVKLSCKASGYTFTSYWINWVKQRPGQGLEWIGNIYPSDSYTNYDQKFKDKATLTVDKSSSTAYMQLSSPTSEDSAVYYCTKSGEYGKIGYYAMDYWGQGTSVTVSSGGCGGGKVAALKEKVAALKEKVAALKEKVAALKE

SEQ ID NO: 114 - protein, 727 aa, synthetic construct
  REGION 1..727: note = Third Polypeptide Chain of DART-G
QVQLVQSGAEVKKPGASVKVSCKASGYTFTNYGMNWVRQAPGQGLEWMGWINTNIGEPTYTEEFKGRVTMTRDTSISTAYMELSRLRSDDTAVYYCARDDGYGNRVSYWGQGTLVTVSSASTKGPSVFPLAPSSKSTSGGTAALGCLVKDYFPEPVTVSWNSGALTSGVHTFPAVLQSSGLYSLSSVVTVPSSSLGTQTYICNVNHKPSNTKVDKRVEPKSCDKTHTCPPCPAPEAAGGPSVFLFPPKPKDTLMISRTPEVTCVVVDVSHEDPEVKFNWYVDGVEVHNAKTKPREEQYNSTYRVVSVLTVLHQDWLNGKEYKCKVSNKALPAPIEKTISKAKGQPREPQVYTLPPSREEMTKNQVSLWCLVKGFYPSDIAVEWESNGQPENNYKTTPPVLDSDGSFFLYSKLTVDKSRWQQGNVFSCSVMHEALHNHYTQKSLSLSPGGGGSGGGSGGGDIQMTQSPSSLSASVGDRVTITCRPSQDISNYLNWYQQKPDKTVKLLIYYTSRLRSGVPSRFSGSGSGTDFTFTISSLQPEDIATYFCQQGDTLPYTFGQGTKLEIKGGGSGGGGQVQLVQSGAEVKKPGASVKVSCKASGYTFTSYWINWVKQAPGQGLEWIGNIYPSDSYTNYNQKFKDKATITADKSTSTAYMELSSLRSEDTAVYYCTRDYGSSYSFDYWGQGTTVTVSSGGCGGGEVAALEKEVAALEKEVAALEKEVAALEK

SEQ ID NO: 115 - protein, 729 aa, synthetic construct
  REGION 1..729: note = Third Polypeptide Chain of Optimized DART-G1
QVQLVQSGAEVKKPGASVKVSCKASGYTFTNYGMNWVRQAPGQGLEWMGWINTNIGEPTYTEEFKGRVTMTRDTSISTAYMELSRLRSDDTAVYYCARDDGYGNRVSYWGQGTLVTVSSASTKGPSVFPLAPSSKSTSGGTAALGCLVKDYFPEPVTVSWNSGALTSGVHTFPAVLQSSGLYSLSSVVTVPSSSLGTQTYICNVNHKPSNTKVDKRVEPKSCDKTHTCPPCPAPEAAGGPSVFLFPPKPKDTLMISRTPEVTCVVVDVSHEDPEVKFNWYVDGVEVHNAKTKPREEQYNSTYRVVSVLTVLHQDWLNGKEYKCKVSNKALPAPIEKTISKAKGQPREPQVYTLPPSREEMTKNQVSLWCLVKGFYPSDIAVEWESNGQPENNYKTTPPVLDSDGSFFLYSKLTVDKSRWQQGNVFSCSVMHEALHNHYTQKSLSLSPGGGGSGGGSGGGDIQMTQSPSSLSASVGDRVTITCRPSQDISNYLNWYQQKPDKTVKLLIYYTSRLRSGVPSRFSGSGSGTDFTFTISSLQPEDIATYFCQQGDTLPYTFGQGTKLEIKGGGSGGGGQVQVQLVQSGAEVKKPGASVKVSCKASGYTFTSYWINWVKQAPGQGLEWIGNIYPSDSYTNYNQKFKDKATITADKSTSTAYMELSSLRSEDTAVYYCTRDYGSAYSFHPWGQGTTVTVSSGGCGGGEVAALEKEVAALEKEVAALEKEVAALEK

SEQ ID NO: 116 - protein, 729 aa, synthetic construct
  REGION 1..729: note = Third Polypeptide Chain of Optimized DART-G2
QVQLVQSGAEVKKPGASVKVSCKASGYTFTNYGMNWVRQAPGQGLEWMGWINTNIGEPTYTEEFKGRVTMTRDTSISTAYMELSRLRSDDTAVYYCARDDGYGNRVSYWGQGTLVTVSSASTKGPSVFPLAPSSKSTSGGTAALGCLVKDYFPEPVTVSWNSGALTSGVHTFPAVLQSSGLYSLSSVVTVPSSSLGTQTYICNVNHKPSNTKVDKRVEPKSCDKTHTCPPCPAPEAAGGPSVFLFPPKPKDTLMISRTPEVTCVVVDVSHEDPEVKFNWYVDGVEVHNAKTKPREEQYNSTYRVVSVLTVLHQDWLNGKEYKCKVSNKALPAPIEKTISKAKGQPREPQVYTLPPSREEMTKNQVSLWCLVKGFYPSDIAVEWESNGQPENNYKTTPPVLDSDGSFFLYSKLTVDKSRWQQGNVFSCSVMHEALHNHYTQKSLSLSPGGGGSGGGSGGGDIQMTQSPSSLSASVGDRVTITCRPSQDISNYLNWYQQKPDKTVKLLIYYTSRLRSGVPSRFSGSGSGTDFTFTISSLQPEDIATYFCQQGDTLPYTFGQGTKLEIKGGGSGGGGQVQVQLVQSGAEVKKPGASVKVSCKASGYTFTSYWINWVKQAPGQGLEWIGNIYPSDSYTNYNQKFKDKATITADKSTSTAYMELSSLRSEDTAVYYCTRDYGSAYSMSTWGQGTTVTVSSGGCGGGEVAALEKEVAALEKEVAALEKEVAALEK

SEQ ID NO: 117 - protein, 729 aa, synthetic construct
  REGION 1..729: note = Third Polypeptide Chain of Optimized DART-G3
QVQLVQSGAEVKKPGASVKVSCKASGYTFTNYGMNWVRQAPGQGLEWMGWINTNIGEPTYTEEFKGRVTMTRDTSISTAYMELSRLRSDDTAVYYCARDDGYGNRVSYWGQGTLVTVSSASTKGPSVFPLAPSSKSTSGGTAALGCLVKDYFPEPVTVSWNSGALTSGVHTFPAVLQSSGLYSLSSVVTVPSSSLGTQTYICNVNHKPSNTKVDKRVEPKSCDKTHTCPPCPAPEAAGGPSVFLFPPKPKDTLMISRTPEVTCVVVDVSHEDPEVKFNWYVDGVEVHNAKTKPREEQYNSTYRVVSVLTVLHQDWLNGKEYKCKVSNKALPAPIEKTISKAKGQPREPQVYTLPPSREEMTKNQVSLWCLVKGFYPSDIAVEWESNGQPENNYKTTPPVLDSDGSFFLYSKLTVDKSRWQQGNVFSCSVMHEALHNHYTQKSLSLSPGGGGSGGGSGGGDIQMTQSPSSLSASVGDRVTITCRPSQDISNYLNWYQQKPDKTVKLLIYYTSRLRSGVPSRFSGSGSGTDFTFTISSLQPEDIATYFCQQGDTLPYTFGQGTKLEIKGGGSGGGGQVQVQLVQSGAEVKKPGASVKVSCKASGYTFTSYWINWVKQAPGQGLEWIGNIYPSDSYTNYNQKFKDKATITADKSTSTAYMELSSLRSEDTAVYYCTRDYGSAYSYSLWGQGTTVTVSSGGCGGGEVAALEKEVAALEKEVAALEKEVAALEK

SEQ ID NO: 118 - protein, 729 aa, synthetic construct
  REGION 1..729: note = Third Polypeptide Chain of Optimized DART-G4
QVQLVQSGAEVKKPGASVKVSCKASGYTFTNYGMNWVRQAPGQGLEWMGWINTNIGEPTYTEEFKGRVTMTRDTSISTAYMELSRLRSDDTAVYYCARDDGYGNRVSYWGQGTLVTVSSASTKGPSVFPLAPSSKSTSGGTAALGCLVKDYFPEPVTVSWNSGALTSGVHTFPAVLQSSGLYSLSSVVTVPSSSLGTQTYICNVNHKPSNTKVDKRVEPKSCDKTHTCPPCPAPEAAGGPSVFLFPPKPKDTLMISRTPEVTCVVVDVSHEDPEVKFNWYVDGVEVHNAKTKPREEQYNSTYRVVSVLTVLHQDWLNGKEYKCKVSNKALPAPIEKTISKAKGQPREPQVYTLPPSREEMTKNQVSLWCLVKGFYPSDIAVEWESNGQPENNYKTTPPVLDSDGSFFLYSKLTVDKSRWQQGNVFSCSVMHEALHNHYTQKSLSLSPGGGGSGGGSGGGDIQMTQSPSSLSASVGDRVTITCRPSQDISNYLNWYQQKPDKTVKLLIYYTSRLRSGVPSRFSGSGSGTDFTFTISSLQPEDIATYFCQQGDTLPYTFGQGTKLEIKGGGSGGGGQVQVQLVQSGAEVKKPGASVKVSCKASGYTFTSYWINWVKQAPGQGLEWIGNIYPSDSYTNYNQKFKDKATITADKSTSTAYMELSSLRSEDTAVYYCTRDYGSSYSYNVWGQGTTVTVSSGGCGGGEVAALEKEVAALEKEVAALEKEVAALEK

SEQ ID NO: 119 - protein, 268 aa, synthetic construct
  REGION 1..268: note = Fourth Polypeptide Chain of DART-G
DIQMTQSPSSLSASVGDRVTITCRPSQDISNYLNWYQQKPDKTVKLLIYYTSRLRSGVPSRFSGSGSGTDFTFTISSLQPEDIATYFCQQGDTLPYTFGQGTKLEIKGGGSGGGGQVQLVQSGAEVKKPGASVKVSCKASGYTFTSYWINWVKQAPGQGLEWIGNIYPSDSYTNYNQKFKDKATITADKSTSTAYMELSSLRSEDTAVYYCTRDYGSSYSFDYWGQGTTVTVSSGGCGGGKVAALKEKVAALKEKVAALKEKVAALKE

SEQ ID NO: 120 - protein, 268 aa, synthetic construct
  REGION 1..268: note = Fourth Polypeptide Chain of Optimized DART-G1
DIQMTQSPSSLSASVGDRVTITCRPSQDISNYLNWYQQKPDKTVKLLIYYTSRLRSGVPSRFSGSGSGTDFTFTISSLQPEDIATYFCQQGDTLPYTFGQGTKLEIKGGGSGGGGQVQLVQSGAEVKKPGASVKVSCKASGYTFTSYWINWVKQAPGQGLEWIGNIYPSDSYTNYNQKFKDKATITADKSTSTAYMELSSLRSEDTAVYYCTRDYGSAYSFHPWGQGTTVTVSSGGCGGGKVAALKEKVAALKEKVAALKEKVAALKE

SEQ ID NO: 121 - protein, 268 aa, synthetic construct
  REGION 1..268: note = Fourth Polypeptide Chain of Optimized DART-G2
DIQMTQSPSSLSASVGDRVTITCRPSQDISNYLNWYQQKPDKTVKLLIYYTSRLRSGVPSRFSGSGSGTDFTFTISSLQPEDIATYFCQQGDTLPYTFGQGTKLEIKGGGSGGGGQVQLVQSGAEVKKPGASVKVSCKASGYTFTSYWINWVKQAPGQGLEWIGNIYPSDSYTNYNQKFKDKATITADKSTSTAYMELSSLRSEDTAVYYCTRDYGSAYSMSTWGQGTTVTVSSGGCGGGKVAALKEKVAALKEKVAALKEKVAALKE

SEQ ID NO: 122 - protein, 268 aa, synthetic construct
  REGION 1..268: note = Fourth Polypeptide Chain of Optimized DART-G3
DIQMTQSPSSLSASVGDRVTITCRPSQDISNYLNWYQQKPDKTVKLLIYYTSRLRSGVPSRFSGSGSGTDFTFTISSLQPEDIATYFCQQGDTLPYTFGQGTKLEIKGGGSGGGGQVQLVQSGAEVKKPGASVKVSCKASGYTFTSYWINWVKQAPGQGLEWIGNIYPSDSYTNYNQKFKDKATITADKSTSTAYMELSSLRSEDTAVYYCTRDYGSAYSYSLWGQGTTVTVSSGGCGGGKVAALKEKVAALKEKVAALKEKVAALKE

SEQ ID NO: 123 - protein, 268 aa, synthetic construct
  REGION 1..268: note = Fourth Polypeptide Chain of Optimized DART-G4
DIQMTQSPSSLSASVGDRVTITCRPSQDISNYLNWYQQKPDKTVKLLIYYTSRLRSGVPSRFSGSGSGTDFTFTISSLQPEDIATYFCQQGDTLPYTFGQGTKLEIKGGGSGGGGQVQLVQSGAEVKKPGASVKVSCKASGYTFTSYWINWVKQAPGQGLEWIGNIYPSDSYTNYNQKFKDKATITADKSTSTAYMELSSLRSEDTAVYYCTRDYGSSYSYNVWGQGTTVTVSSGGCGGGKVAALKEKVAALKEKVAALKEKVAALKE

SEQ ID NO: 124 - protein, 118 aa, Mus musculus
  REGION 1..118: note = MISC_FEATURE - VH Domain of Anti-Fluorescein Antibody 4-4-20
EVKLDETGGGLVQPGRPMKLSCVASGFTFSDYWMNWVRQSPEKGLEWVAQIRNKPYNYETYYSDSVKGRFTISRDDSKSSVYLQMNNLRVEDMGIYYCTGSYYGMDYWGQGTSVTVSS

SEQ ID NO: 125 - protein, 112 aa, Mus musculus
  REGION 1..112: note = MISC_FEATURE - VL Domain of Anti-Fluorescein Antibody 4-4-20
DVVMTQTPFSLPVSLGDQASISCRSSQSLVHSNGNTYLRWYLQKPGQSPKVLIYKVSNRFSGVPDRFSGSGSGTDFTLKISRVEAEDLGVYFCSQSTHVPWTFGGGTKLEIK

SEQ ID NO: 126 - protein, 120 aa, synthetic construct
  REGION 1..120: note = VH Domain of Palivizumab
QVTLRESGPALVKPTQTLTLTCTFSGFSLSTSGMSVGWIRQPPGKALEWLADIWWDDKKDYNPSLKSRLTISKDTSKNQVVLKVTNMDPADTATYYCARSMITNWYFDVWGAGTTVTVSS

SEQ ID NO: 127 - protein, 106 aa, synthetic construct
  REGION 1..106: note = VL Domain of Palivizumab
DIQMTQSPSTLSASVGDRVTITCRASQSVGYMHWYQQKPGKAPKLLIYDTSKLASGVPSRFSGSGSGTEFTLTISSLQPDDFATYYCFQGSGYPFTFGGGTKLEIK

SEQ ID NO: 128 - protein, 118 aa, Mus musculus
  REGION 1..118: note = MISC_FEATURE - VH Domain of EphA2 MAB-1
QVQLKESGPGLVAPSQSLSITCTVSGFSLSRYSVHWVRQPPGKGLEWLGMIWGGGSTDYNSALKSRLSISKDNSKSQVFLKMNSLQTDDTAMYYCARKHGNYYTMDYWGQGTSVTVSS

SEQ ID NO: 129 - protein, 106 aa, Mus musculus
  REGION 1..106: note = MISC_FEATURE - VL Domain of EphA2 MAB-1
DIQMTQTTSSLSASLGDRITISCRASQDISNYLNWYQQKPDGTVKLLIYYTSRLHSGVPSRFSGSGSGTDYSLTISNLEQEDIATYFCQQGYTLYTFGGGTKLEIK

SEQ ID NO: 130 - protein, 118 aa, Mus musculus
  REGION 1..118: note = MISC_FEATURE - VH Domain of EphA2 MAB-2
QIQLVQSGPELKKPGETVKISCKASGFTFTNYGMNWVKQAPGKGLKWMGWINTYIGEPTYADDFKGRFVFSLETSASTAYLQINNLKNEDMATYFCARELGPYYFDYWGQGTTLTVSS

SEQ ID NO: 131 - protein, 111 aa, Mus musculus
  REGION 1..111: note = MISC_FEATURE - VL Domain of EphA2 MAB-2
DVVMTQTPLSLPVSLGDQASISCRSSQSLVHSSGNTYLHWYLQKPGQSPKLLIYKVSNRFSGVPDRFSGSGSGTDFTLKISRVEAEDLGVYFCSQSTHVPTFGSGTKLEIK

SEQ ID NO: 132 - protein, 118 aa, Mus musculus
  REGION 1..118: note = MISC_FEATURE - VH Domain of EphA2 MAB-3
EVQLVESGGGSVKPGGSLKLSCAASGFTFTDHYMYWVRQTPEKRLEWVATISDGGSFTSYPDSVKGRFTISRDIAKNNLYLQMSSLKSEDTAMYYCTRDESDRPFPYWGQGTLVTVSS

SEQ ID NO: 133 - protein, 107 aa, Mus musculus
  REGION 1..107: note = MISC_FEATURE - VL Domain of EphA2 MAB-3
DIVLTQSHRSMSTSVGDRVNITCKASQDVTTAVAWYQQKPGQSPKLLIFWASTRHAGVPDRFTGSGSGTDFTLTISSVQAGDLALYYCQQHYSTPYTFGGGTKLEIK

SEQ ID NO: 134 - protein, 118 aa, Mus musculus
  REGION 1..118: note = MISC_FEATURE - VH Domain of 5T4 MAB-1
QVQLVQSGAEVKKPGASVKVSCKASGYTFTSFWMHWVRQAPGQGLEWMGRIDPNRGGTEYNEKAKSRVTMTADKSTSTAYMELSSLRSEDTAVYYCAGGNPYYPMDYWGQGTTVTVSS

SEQ ID NO: 135 - protein, 107 aa, Mus musculus
  REGION 1..107: note = MISC_FEATURE - VL Domain of 5T4 MAB-1
DIQMTQSPSSLSASVGDRVTITCRASQGISNYLAWFQQKPGKAPKSLIYRANRLQSGVPSRFSGSGSGTDFTLTISSLQPEDVATYYCLQYDDFPWTFGQGTKLEIK

SEQ ID NO: 136 - protein, 127 aa, Mus musculus
  REGION 1..127: note = MISC_FEATURE - VH Domain of 5T4 MAB-2
QVQLQQPGAELVKPGASVKMSCKASGYTFTSYWITWVKQRPGQGLEWIGDIYPGSGRANYNEKFKSKATLTVDTSSSTAYMQLSSLTSEDSAVYNCARYGPLFTTVVDPNSYAMDYWGQGTSVTVSS

SEQ ID NO: 137 - protein, 112 aa, Mus musculus
  REGION 1..112: note = MISC_FEATURE - VL Domain of 5T4 MAB-2
DVLMTQTPLSLPVSLGDQASISCRSSQSIVYSNGNTYLEWYLQKPGQSPKLLIYKVSNRFSGVPDRFSGSGSGTDFTLKISRVEAEDLGVYYCFQGSHVPFTFGSGTKLEIK

SEQ ID NO: 138 - protein, 122 aa, synthetic construct
  REGION 1..122: note = VH Domain of Fc-Optimized Anti-Human B7-H3 Antibody Enoblituzumab
EVQLVESGGGLVQPGGSLRLSCAASGFTFSSFGMHWVRQAPGKGLEWVAYISSDSSAIYYADTVKGRFTISRDNAKNSLYLQMNSLRDEDTAVYYCGRGRENIYYGSRLDYWGQGTTVTVSS

SEQ ID NO: 139 - protein, 107 aa, synthetic construct
  REGION 1..107: note = VL Domain of Fc-Optimized Anti-Human B7-H3 Antibody Enoblituzumab
DIQLTQSPSFLSASVGDRVTITCKASQNVDTNVAWYQQKPGKAPKALIYSASYRYSGVPSRFSGSGSGTDFTLTISSLQPEDFATYYCQQYNNYPFTFGQGTKLEIK

SEQ ID NO: 140 - protein, 120 aa, Mus musculus
  REGION 1..120: note = MISC_FEATURE - VH Domain of Anti-Human B7-H3 Antibody BRCA69D
QVQLQQSGAELARPGASVKLSCKASGYTFTSYWMQWVKQRPGQGLEWIGTIYPGDGDTRYTQKFKGKATLTADKSSSTAYMQLSSLASEDSAVYYCARRGIPRLWYFDVWGAGTTVTVSS

SEQ ID NO: 141 - protein, 107 aa, Mus musculus
  REGION 1..107: note = MISC_FEATURE - VL Domain of Anti-Human B7-H3 Antibody BRCA69D
DIQMTQTTSSLSASLGDRVTISCRASQDISNYLNWYQQKPDGTVKLLIYYTSRLHSGVPSRFSGSGSGTDYSLTIDNLEQEDIATYFCQQGNTLPPTFGGGTKLEIK

SEQ ID NO: 142 - protein, 120 aa, synthetic construct
  REGION 1..120: note = VH Domain of Humanized Anti-Human B7-H3 Antibody BRCA69D (hBRCA69D VH1)
QVQLVQSGAEVKKPGASVKVSCKASGYTFTSYWMQWVRQAPGQGLEWMGTIYPGDGDTRYTQKFKGRVTITADKSTSTAYMELSSLRSEDTAVYYCARRGIPRLWYFDVWGQGTTVTVSS

SEQ ID NO: 143 - protein, 120 aa, synthetic construct
  REGION 1..120: note = VH Domain of Humanized Anti-Human B7-H3 Antibody BRCA69D (hBRCA69D VH2)
QVQLVQSGAEVKKPGASVKVSCKASGYTFTSYWMQWVRQAPGQGLEWMGTIYPGGGDTRYTQKFQGRVTITADKSTSTAYMELSSLRSEDTAVYYCARRGIPRLWYFDVWGQGTTVTVSS

SEQ ID NO: 144 - protein, 107 aa, synthetic construct
  REGION 1..107: note = VL Domain of Humanized Anti-Human B7-H3 Antibody BRCA69D (hBRCA69D VL1)
DIQMTQSPSSLSASVGDRVTITCRASQDISNYLNWYQQKPGKAPKLLIYYTSRLHSGVPSRFSGSGSGTDFTLTISSLQPEDIATYYCQQGNTLPPTFGGGTKLEIK

SEQ ID NO: 145 - protein, 107 aa, synthetic construct
  REGION 1..107: note = VL Domain of Humanized Anti-Human B7-H3 Antibody BRCA69D (hBRCA69D VL2)
DIQMTQSPSSLSASVGDRVTITCRASQSISSYLNWYQQKPGKAPKLLIYYTSRLQSGVPSRFSGSGSGTDFTLTISSLQPEDIATYYCQQGNTLPPTFGGGTKLEIK

SEQ ID NO: 146 - protein, 117 aa, Mus musculus
  REGION 1..117: note = MISC_FEATURE - VH Domain of Anti-Human B7-H3 Antibody PRCA157
EVQQVESGGDLVKPGGSLKLSCAASGFTFSSYGMSWVRQTPDKRLEWVATINSGGSNTYYPDSLKGRFTISRDNAKNTLYLQMRSLKSEDTAMYYCARHDGGAMDYWGQGTSVTVSS

SEQ ID NO: 147 - protein, 108 aa, Mus musculus
  REGION 1..108: note = MISC_FEATURE - VL Domain of Anti-Human B7-H3 Antibody PRCA157
DIQMTQSPASLSVSVGETVTITCRASESIYSYLAWYQQKQGKSPQLLVYNTKTLPEGVPSRFSGSGSGTQFSLKINSLQPEDFGRYYCQHHYGTPPWTFGGGTNLEIK

SEQ ID NO: 148 - protein, 119 aa, Mus musculus
  REGION 1..119: note = MISC_FEATURE - VH Domain of Anti-gpA33 Antibody gpA33 MAB-1
QVQLVQSGAEVKKPGASVKVSCKASGYTFTGSWMNWVRQAPGQGLEWIGRIYPGDGETNYNGKFKDRVTITADKSTSTAYMELSSLRSEDTAVYYCARIYGNNVYFDVWGQGTTVTVSS

SEQ ID NO: 149 - protein, 106 aa, Mus musculus
  REGION 1..106: note = MISC_FEATURE - VL Domain of Anti-gpA33 Antibody gpA33 MAB-1
DIQLTQSPSFLSASVGDRVTITCSARSSISFMYWYQQKPGKAPKLLIYDTSNLASGVPSRFSGSGSGTEFTLTISSLEAEDAATYYCQQWSSYPLTFGQGTKLEIK

SEQ ID NO: 150 - protein, 121 aa, synthetic construct
  REGION 1..121: note = VH Domain of Humanized Anti-CEACAM5/CEACAM6 Antibody 16C3
QVQLQQSGPEVVRPGVSVKISCKGSGYTFTDYAMHWVKQSHAKSLEWIGLISTYSGDTKYNQNFKGKATMTVDKSASTAYMELSSLRSEDTAVYYCARGDYSGSRYWFAYWGQGTLVTVSS

SEQ ID NO: 151 - protein, 107 aa, synthetic construct
  REGION 1..107: note = VL Domain of Humanized Anti-CEACAM5/CEACAM6 Antibody 16C3
DIQMTQSPSSLSASVGDRVTITCGASENIYGALNWYQRKPGKSPKLLIWGASNLADGMPSRFSGSGSGRQYTLTISSLQPEDVATYYCQNVLSSPYTFGGGTKLEIK

SEQ ID NO: 152 - protein, 121 aa, synthetic construct
  REGION 1..121: note = VH Domain of Humanized Anti-CEACAM5/CEACAM6 Antibody hMN15
QVQLVESGGGVVQPGRSLRLSCSSSGFALTDYYMSWVRQAPGKGLEWLGFIANKANGHTTDYSPSVKGRFTISRDNSKNTLFLQMDSLRPEDTGVYFCARDMGIRWNFDVWGQGTPVTVSS

SEQ ID NO: 153 - protein, 107 aa, synthetic construct
  REGION 1..107: note = VL Domain of Humanized Anti-CEACAM5/CEACAM6 Antibody hMN15
DIQLTQSPSSLSASVGDRVTMTCSASSRVSYIHWYQQKPGKAPKRWIYGTSTLASGVPARFSGSGSGTDFTFTISSLQPEDIATYYCQQWSYNPPTFGQGTKVEIKR

SEQ ID NO: 154 - protein, 5 aa, Mus musculus
  REGION 1..5: note = MISC_FEATURE - CDRH1 of Murine Anti-CD137 Monoclonal Antibody (CD137 MAB-3 VH)
SYWIN

SEQ ID NO: 155 - protein, 17 aa, Mus musculus
  REGION 1..17: note = MISC_FEATURE - CDRH2 of Murine Anti-CD137 Monoclonal Antibody (CD137 MAB-3 VH)
NIYPSDSYTNYNQKFKD

SEQ ID NO: 156 - protein, 10 aa, Mus musculus
  REGION 1..10: note = MISC_FEATURE - CDRH3 of Murine Anti-CD137 Monoclonal Antibody (CD137 MAB-3 VH)
DYGSSYSFDY

SEQ ID NO: 157 - protein, 11 aa, Mus musculus
  REGION 1..11: note = MISC_FEATURE - CDRL1 of Murine Anti-CD137 Monoclonal Antibody (CD137 MAB-3 VL)
RPSQDISNYLN

SEQ ID NO: 158 - protein, 7 aa, Mus musculus
  REGION 1..7: note = MISC_FEATURE - CDRL2 of Murine Anti-CD137 Monoclonal Antibody (CD137 MAB-3 VL)
YTSRLRS

SEQ ID NO: 159 - protein, 9 aa, Mus musculus
  REGION 1..9: note = MISC_FEATURE - CDRL3 of Murine Anti-CD137 Monoclonal Antibody (CD137 MAB-3 VL)
QQGDTLPYT

SEQ ID NO: 160 - protein, 6 aa, Mus musculus
  REGION 1..6: note = 1MISC_FEATURE - Residues 103-108 of SEQ ID NO:74
SYSFDY

SEQ ID NO: 161 - protein, 10 aa, synthetic construct
  REGION 1..10: note = CDRH3 of hCD137 MAB-3 VH1A
DYGSAYSFHP

SEQ ID NO: 162 - protein, 10 aa, synthetic construct
  REGION 1..10: note = CDRH3 of hCD137 MAB-3 VH1B
DYGSAYSMST

SEQ ID NO: 163 - protein, 10 aa, synthetic construct
  REGION 1..10: note = CDRH3 of hCD137 MAB-3 VH1C
DYGSAYSYSL

SEQ ID NO: 164 - protein, 10 aa, synthetic construct
  REGION 1..10: note = CDRH3 of hCD137 MAB-3 VH1D
DYGSSYSYNV

SEQ ID NO: 165 - protein, 5 aa, Mus musculus
  REGION 1..5: note = MISC_FEATURE - CDRH1 of CD137 MAB-4 VH
SYWIN

SEQ ID NO: 166 - protein, 17 aa, Mus musculus
  REGION 1..17: note = MISC_FEATURE - CDRH2 of CD137 MAB-4 VH
NIYPSDSYTNYDQKFKD

SEQ ID NO: 167 - protein, 14 aa, Mus musculus
  REGION 1..14: note = MISC_FEATURE - CDRH3 of CD137 MAB-4 VH
SGEYGKIGYYAMDY

SEQ ID NO: 168 - protein, 11 aa, Mus musculus
  REGION 1..11: note = MISC_FEATURE - CDRL1 of CD137 MAB-4 VL
RASQDISNYLN

SEQ ID NO: 169 - protein, 7 aa, Mus musculus
  REGION 1..7: note = MISC_FEATURE - CDRL2 of CD137 MAB-4 VL
YTSRLHS

SEQ ID NO: 170 - protein, 9 aa, Mus musculus
  REGION 1..9: note = MISC_FEATURE - CDRL3 of CD137 MAB-4 VL
QQGNTLPYT

SEQ ID NO: 171 - protein, 5 aa, Mus musculus
  REGION 1..5: note = MISC_FEATURE - CDRH1 of CD137 MAB-5 VH
SYDIS

SEQ ID NO: 172 - protein, 16 aa, Mus musculus
  REGION 1..16: note = MISC_FEATURE - CDRH2 of CD137 MAB-5 VH
VVWTGGGTNYNSAFMS

SEQ ID NO: 173 - skipped

SEQ ID NO: 174 - protein, 16 aa, Mus musculus
  REGION 1..16: note = MISC_FEATURE - CDRL1 of CD137 MAB-5 VL
RSSQSLVHSNGNTYLH

SEQ ID NO: 175 - protein, 7 aa, Mus musculus
  REGION 1..7: note = MISC_FEATURE - CDRL2 of CD137 MAB-5 VL
KVSNRFS

SEQ ID NO: 176 - protein, 9 aa, Mus musculus
  REGION 1..9: note = MISC_FEATURE - CDRL3 of CD137 MAB-5 VL
SQSTHVPWT

SEQ ID NO: 177 - protein, 5 aa, Mus musculus
  REGION 1..5: note = MISC_FEATURE - CDRH1 of Murine Anti-HER2/neu Monoclonal Antibody HER2 MAB-1 VH
NYGMN

SEQ ID NO: 178 - protein, 17 aa, Mus musculus
  REGION 1..17: note = MISC_FEATURE - CDRH2 of Murine Anti-HER2/neu Monoclonal Antibody HER2 MAB-1 VH
WINTNIGEPTYTEEFKG

SEQ ID NO: 179 - protein, 10 aa, Mus musculus
  REGION 1..10: note = MISC_FEATURE - CDRH3 of Murine Anti-HER2/neu Monoclonal Antibody HER2 MAB-1 VH
DDGYGNRVSY

SEQ ID NO: 180 - protein, 11 aa, Mus musculus
  REGION 1..11: note = MISC_FEATURE - CDRL1 of Murine Anti-HER2/neu Monoclonal Antibody HER2 MAB-1 VL
KASQDINSYLS

SEQ ID NO: 181 - protein, 7 aa, Mus musculus
  REGION 1..7: note = MISC_FEATURE - CDRL2 of Murine Anti-HER2/neu Monoclonal Antibody HER2 MAB-1 VL
RANRLVD

SEQ ID NO: 182 - protein, 9 aa, Mus musculus
  REGION 1..9: note = MISC_FEATURE - CDRL3 of Murine Anti-HER2/neu Monoclonal Antibody HER2 MAB-1 VL
LQHDEFPWT

SEQ ID NO: 183 - protein, 10 aa, synthetic construct
  REGION 1..10: note = CDRH3 of VH Domain of Humanized Anti-Human HER2/neu Antibody (hHER2 MAB-1 VH1)
DDGYGNRVSY

SEQ ID NO: 184 - protein, 10 aa, synthetic construct
  REGION 1..10: note = CDRH3 of VH Domain of Humanized Anti-Human HER2/neu Antibody (hHER2 MAB-1 VH2)
DEGYGNRVSY

SEQ ID NO: 185 - protein, 10 aa, synthetic construct
  REGION 1..10: note = CDRH3 of VH Domain of Humanized Anti-Human HER2/neu Antibody (hHER2 MAB-1 VH3)
DDIYGNRVSY

SEQ ID NO: 186 - protein, 11 aa, synthetic construct
  REGION 1..11: note = CDRL1 of VL Domain of Humanized Anti-Human HER2/neu Antibody (hHER2 MAB-1 VL1)
KASQDINSYLS

SEQ ID NO: 187 - protein, 11 aa, synthetic construct
  REGION 1..11: note = CDRL1 of VL Domain of Humanized Anti-Human HER2/neu Antibody (hHER2 MAB-1 VL2)
KASQDINTYLS

SEQ ID NO: 188 - protein, 11 aa, synthetic construct
  REGION 1..11: note = CDRL1 of VL Domain of Humanized Anti-Human HER2/neu Antibody (hHER2 MAB-1 VL3)
KASQDISNYLS

SEQ ID NO: 189 - protein, 7 aa, synthetic construct
  REGION 1..7: note = CDRL2 of VL Domain of Humanized Anti-Human HER2/neu Antibody (hHER2 MAB-1 VL1)
RANRLVD

SEQ ID NO: 190 - protein, 7 aa, synthetic construct
  REGION 1..7: note = CDRL2 of VL Domain of Humanized Anti-Human HER2/neu Antibody (hHER2 MAB-1 VL2)
RANRLVE

SEQ ID NO: 191 - protein, 7 aa, synthetic construct
  REGION 1..7: note = CDRL2 of VL Domain of Humanized Anti-Human HER2/neu Antibody (hHER2 MAB-1 VL3)
RANRLQS

SEQ ID NO: 192 - protein, 497 aa, synthetic construct
  REGION 1..497: note = First Polypeptide Chain of TRIDENT-A
DIQMTQSPSSLSASVGDRVTITCRPSQDISNYLNWYQQKPDKTVKLLIYYTSRLRSGVPSRFSGSGSGTDFTFTISSLQPEDIATYFCQQGDTLPYTFGQGTKLEIKGGGSGGGGQVQLVQSGAEVKKPGASVKVSCKASGYTFTSYWINWVKQAPGQGLEWIGNIYPSDSYTNYNQKFKDKATITADKSTSTAYMELSSLRSEDTAVYYCTRDYGSSYSFDYWGQGTTVTVSSASTKGEVAACEKEVAALEKEVAALEKEVAALEKGGGDKTHTCPPCPAPEAAGGPSVFLFPPKPKDTLMISRTPEVTCVVVDVSHEDPEVKFNWYVDGVEVHNAKTKPREEQYNSTYRVVSVLTVLHQDWLNGKEYKCKVSNKALPAPIEKTISKAKGQPREPQVYTLPPSREEMTKNQVSLWCLVKGFYPSDIAVEWESNGQPENNYKTTPPVLDSDGSFFLYSKLTVDKSRWQQGNVFSCSVMHEALHNHYTQKSLSLSPGK

SEQ ID NO: 193 - protein, 497 aa, synthetic construct
  REGION 1..497: note = First Polypeptide Chain of TRIDENT-A1
DIQMTQSPSSLSASVGDRVTITCRPSQDISNYLNWYQQKPDKTVKLLIYYTSRLRSGVPSRFSGSGSGTDFTFTISSLQPEDIATYFCQQGDTLPYTFGQGTKLEIKGGGSGGGGQVQLVQSGAEVKKPGASVKVSCKASGYTFTSYWINWVKQAPGQGLEWIGNIYPSDSYTNYNQKFKDKATITADKSTSTAYMELSSLRSEDTAVYYCTRDYGSAYSFHPWGQGTTVTVSSASTKGEVAACEKEVAALEKEVAALEKEVAALEKGGGDKTHTCPPCPAPEAAGGPSVFLFPPKPKDTLMISRTPEVTCVVVDVSHEDPEVKFNWYVDGVEVHNAKTKPREEQYNSTYRVVSVLTVLHQDWLNGKEYKCKVSNKALPAPIEKTISKAKGQPREPQVYTLPPSREEMTKNQVSLWCLVKGFYPSDIAVEWESNGQPENNYKTTPPVLDSDGSFFLYSKLTVDKSRWQQGNVFSCSVMHEALHNHYTQKSLSLSPGK

SEQ ID NO: 194 - protein, 497 aa, synthetic construct
  REGION 1..497: note = First Polypeptide Chain of TRIDENT-A2
DIQMTQSPSSLSASVGDRVTITCRPSQDISNYLNWYQQKPDKTVKLLIYYTSRLRSGVPSRFSGSGSGTDFTFTISSLQPEDIATYFCQQGDTLPYTFGQGTKLEIKGGGSGGGGQVQLVQSGAEVKKPGASVKVSCKASGYTFTSYWINWVKQAPGQGLEWIGNIYPSDSYTNYNQKFKDKATITADKSTSTAYMELSSLRSEDTAVYYCTRDYGSAYSMSTWGQGTTVTVSSASTKGEVAACEKEVAALEKEVAALEKEVAALEKGGGDKTHTCPPCPAPEAAGGPSVFLFPPKPKDTLMISRTPEVTCVVVDVSHEDPEVKFNWYVDGVEVHNAKTKPREEQYNSTYRVVSVLTVLHQDWLNGKEYKCKVSNKALPAPIEKTISKAKGQPREPQVYTLPPSREEMTKNQVSLWCLVKGFYPSDIAVEWESNGQPENNYKTTPPVLDSDGSFFLYSKLTVDKSRWQQGNVFSCSVMHEALHNHYTQKSLSLSPGK

SEQ ID NO: 195 - protein, 497 aa, synthetic construct
  REGION 1..497: note = First Polypeptide Chain of TRIDENT-A3
DIQMTQSPSSLSASVGDRVTITCRPSQDISNYLNWYQQKPDKTVKLLIYYTSRLRSGVPSRFSGSGSGTDFTFTISSLQPEDIATYFCQQGDTLPYTFGQGTKLEIKGGGSGGGGQVQLVQSGAEVKKPGASVKVSCKASGYTFTSYWINWVKQAPGQGLEWIGNIYPSDSYTNYNQKFKDKATITADKSTSTAYMELSSLRSEDTAVYYCTRDYGSAYSYSLWGQGTTVTVSSASTKGEVAACEKEVAALEKEVAALEKEVAALEKGGGDKTHTCPPCPAPEAAGGPSVFLFPPKPKDTLMISRTPEVTCVVVDVSHEDPEVKFNWYVDGVEVHNAKTKPREEQYNSTYRVVSVLTVLHQDWLNGKEYKCKVSNKALPAPIEKTISKAKGQPREPQVYTLPPSREEMTKNQVSLWCLVKGFYPSDIAVEWESNGQPENNYKTTPPVLDSDGSFFLYSKLTVDKSRWQQGNVFSCSVMHEALHNHYTQKSLSLSPGK

SEQ ID NO: 196 - protein, 497 aa, synthetic construct
  REGION 1..497: note = First Polypeptide Chain of TRIDENT-A4
DIQMTQSPSSLSASVGDRVTITCRPSQDISNYLNWYQQKPDKTVKLLIYYTSRLRSGVPSRFSGSGSGTDFTFTISSLQPEDIATYFCQQGDTLPYTFGQGTKLEIKGGGSGGGGQVQLVQSGAEVKKPGASVKVSCKASGYTFTSYWINWVKQAPGQGLEWIGNIYPSDSYTNYNQKFKDKATITADKSTSTAYMELSSLRSEDTAVYYCTRDYGSSYSYNVWGQGTTVTVSSASTKGEVAACEKEVAALEKEVAALEKEVAALEKGGGDKTHTCPPCPAPEAAGGPSVFLFPPKPKDTLMISRTPEVTCVVVDVSHEDPEVKFNWYVDGVEVHNAKTKPREEQYNSTYRVVSVLTVLHQDWLNGKEYKCKVSNKALPAPIEKTISKAKGQPREPQVYTLPPSREEMTKNQVSLWCLVKGFYPSDIAVEWESNGQPENNYKTTPPVLDSDGSFFLYSKLTVDKSRWQQGNVFSCSVMHEALHNHYTQKSLSLSPGK

SEQ ID NO: 197 - protein, 267 aa, synthetic construct
  REGION 1..267: note = Second Polypeptide Chain of TRIDENT-A
DIQMTQSPSSLSASVGDRVTITCRPSQDISNYLNWYQQKPDKTVKLLIYYTSRLRSGVPSRFSGSGSGTDFTFTISSLQPEDIATYFCQQGDTLPYTFGQGTKLEIKGGGSGGGGQVQLVQSGAEVKKPGASVKVSCKASGYTFTSYWINWVKQAPGQGLEWIGNIYPSDSYTNYNQKFKDKATITADKSTSTAYMELSSLRSEDTAVYYCTRDYGSSYSFDYWGQGTTVTVSSASTKGKVAACKEKVAALKEKVAALKEKVAALKE

SEQ ID NO: 198 - protein, 267 aa, synthetic construct
  REGION 1..267: note = Second Polypeptide Chain of TRIDENT-A1
DIQMTQSPSSLSASVGDRVTITCRPSQDISNYLNWYQQKPDKTVKLLIYYTSRLRSGVPSRFSGSGSGTDFTFTISSLQPEDIATYFCQQGDTLPYTFGQGTKLEIKGGGSGGGGQVQLVQSGAEVKKPGASVKVSCKASGYTFTSYWINWVKQAPGQGLEWIGNIYPSDSYTNYNQKFKDKATITADKSTSTAYMELSSLRSEDTAVYYCTRDYGSAYSFHPWGQGTTVTVSSASTKGKVAACKEKVAALKEKVAALKEKVAALKE

SEQ ID NO: 199 - protein, 267 aa, synthetic construct
  REGION 1..267: note = Second Polypeptide Chain of TRIDENT-A2
DIQMTQSPSSLSASVGDRVTITCRPSQDISNYLNWYQQKPDKTVKLLIYYTSRLRSGVPSRFSGSGSGTDFTFTISSLQPEDIATYFCQQGDTLPYTFGQGTKLEIKGGGSGGGGQVQLVQSGAEVKKPGASVKVSCKASGYTFTSYWINWVKQAPGQGLEWIGNIYPSDSYTNYNQKFKDKATITADKSTSTAYMELSSLRSEDTAVYYCTRDYGSAYSMSTWGQGTTVTVSSASTKGKVAACKEKVAALKEKVAALKEKVAALKE

SEQ ID NO: 200 - protein, 267 aa, synthetic construct
  REGION 1..267: note = Second Polypeptide Chain of TRIDENT-A3
DIQMTQSPSSLSASVGDRVTITCRPSQDISNYLNWYQQKPDKTVKLLIYYTSRLRSGVPSRFSGSGSGTDFTFTISSLQPEDIATYFCQQGDTLPYTFGQGTKLEIKGGGSGGGGQVQLVQSGAEVKKPGASVKVSCKASGYTFTSYWINWVKQAPGQGLEWIGNIYPSDSYTNYNQKFKDKATITADKSTSTAYMELSSLRSEDTAVYYCTRDYGSAYSYSLWGQGTTVTVSSASTKGKVAACKEKVAALKEKVAALKEKVAALKE

SEQ ID NO: 201 - protein, 267 aa, synthetic construct
  REGION 1..267: note = Second Polypeptide Chain of TRIDENT-A4
DIQMTQSPSSLSASVGDRVTITCRPSQDISNYLNWYQQKPDKTVKLLIYYTSRLRSGVPSRFSGSGSGTDFTFTISSLQPEDIATYFCQQGDTLPYTFGQGTKLEIKGGGSGGGGQVQLVQSGAEVKKPGASVKVSCKASGYTFTSYWINWVKQAPGQGLEWIGNIYPSDSYTNYNQKFKDKATITADKSTSTAYMELSSLRSEDTAVYYCTRDYGSSYSYNVWGQGTTVTVSSASTKGKVAACKEKVAALKEKVAALKEKVAALKE

SEQ ID NO: 202 - protein, 117 aa, synthetic construct
  REGION 1..117: note = VH Domain of hPRCA157 VH1
EVQLVESGGGLVKPGGSLRLSCAASGFTFSSYGMSWVRQAPGKGLEWVATINSGGSNTYYPDSLKGRFTISRDNAKNSLYLQMNSLRAEDTAVYYCARHDGGAMDYWGQGTTVTVSS

SEQ ID NO: 203 - protein, 108 aa, synthetic construct
  REGION 1..108: note = VL Domain of hPRCA157 VL1
DIQMTQSPSSLSASVGDRVTITCRASESIYSYLAWYQQKPGKAPKLLVYNTKTLPEGVPSRFSGSGSGTDFTLTISSLQPEDFATYYCQHHYGTPPWTFGQGTRLEIK

SEQ ID NO: 204 - protein, 120 aa, Mus musculus
  REGION 1..120: note = MISC_FEATURE - VH Domain of CD19 MAB-1
QVTLRESGPALVKPTQTLTLTCTFSGFSLSTSGMGVGWIRQPPGKALEWLAHIWWDDDKRYNPALKSRLTISKDTSKNQVFLTMTNMDPVDTATYYCARMELWSYYFDYWGQGTTVTVSS

SEQ ID NO: 205 - protein, 106 aa, Mus musculus
  REGION 1..106: note = MISC_FEATURE - VL Domain of CD19 MAB-1
ENVLTQSPATLSVTPGEKATITCRASQSVSYMHWYQQKPGQAPRLLIYDASNRASGVPSRFSGSGSGTDHTLTISSLEAEDAATYYCFQGSVYPFTFGQGTKLEIK

SEQ ID NO: 206 - protein, 120 aa, Mus musculus
  REGION 1..120: note = MISC_FEATURE - VH Domain of CD123 MAB-1
EVQLVQSGAELKKPGASVKVSCKASGYTFTDYYMKWVRQAPGQGLEWIGDIIPSNGATFYNQKFKGRVTITVDKSTSTAYMELSSLRSEDTAVYYCARSHLLRASWFAYWGQGTLVTVSS

SEQ ID NO: 207 - protein, 113 aa, Mus musculus
  REGION 1..113: note = MISC_FEATURE - VL Domain of CD123 MAB-1
DFVMTQSPDSLAVSLGERVTMSCKSSQSLLNSGNQKNYLTWYQQKPGQPPKLLIYWASTRESGVPDRFSGSGSGTDFTLTISSLQAEDVAVYYCQNDYSYPYTFGQGTKLEIK

SEQ ID NO: 208 - protein, 119 aa, synthetic construct
  REGION 1..119: note = VH Domain oif of hCD137 MAB-3 VH1E
QVQLVQSGAEVKKPGASVKVSCKASGYTFTSYWINWVRQAPGQGLEWIGNIYPSDSYTNYNQKFKDKATITADKSTSTAYMELSSLRSEDTAVYYCTRDYGSAYSMSTWGQGTTVTVSS

SEQ ID NO: 209 - protein, 119 aa, synthetic construct
  REGION 1..119: note = VH Domain oif of hCD137 MAB-3 VH1F
QVQLVQSGAEVKKPGASVKVSCKASGYTFTSYWINWVKQAPGQGLEWAGNIYPSDSYTNYNQKFKDKATITADKSTSTAYMELSSLRSEDTAVYYCTRDYGSAYSMSTWGQGTTVTVSS

SEQ ID NO: 210 - protein, 119 aa, synthetic construct
  REGION 1..119: note = VH Domain oif of hCD137 MAB-3 VH1G
QVQLVQSGAEVKKPGASVKVSCKASGYTFTSYWINWVRQAPGQGLEWAGNIYPSDSYTNYNQKFKDKATITADKSTSTAYMELSSLRSEDTAVYYCTRDYGSAYSMSTWGQGTTVTVSS

SEQ ID NO: 211 - protein, 107 aa, synthetic construct
  REGION 1..107: note = VL Domain oif of hCD137 MAB-3 VL4
DIQMTQSPSSLSASVGDRVTITCQASQDISNYLNWYQQKPDKTVKLLIYYTSRLRSGVPSRFSGSGSGTDFTFTISSLQPEDIATYFCQQGDTLPYTFGQGTKLEIK

SEQ ID NO: 212 - protein, 107 aa, synthetic construct
  REGION 1..107: note = VL Domain oif of hCD137 MAB-3 VL5
DIQMTQSPSSLSASVGDRVTITCRPSQDISNYLNWYQQKPDKTAKLLIYYTSRLRSGVPSRFSGSGSGTDFTFTISSLQPEDIATYFCQQGDTLPYTFGQGTKLEIK

SEQ ID NO: 213 - protein, 107 aa, synthetic construct
  REGION 1..107: note = VL Domain oif of hCD137 MAB-3 VL6
DIQMTQSPSSLSASVGDRVTITCRPSQDISNYLNWYQQKPDKTVKLLIYYTSRARSGVPSRFSGSGSGTDFTFTISSLQPEDIATYFCQQGDTLPYTFGQGTKLEIK

SEQ ID NO: 214 - protein, 107 aa, synthetic construct
  REGION 1..107: note = VL Domain oif of hCD137 MAB-3 VL7
DIQMTQSPSSLSASVGDRVTITCQASQDISNYLNWYQQKPDKTAKLLIYYTSRLRSGVPSRFSGSGSGTDFTFTISSLQPEDIATYFCQQGDTLPYTFGQGTKLEIK

SEQ ID NO: 215 - protein, 107 aa, synthetic construct
  REGION 1..107: note = VL Domain oif of hCD137 MAB-3 VL8
DIQMTQSPSSLSASVGDRVTITCQASQDISNYLNWYQQKPDKTAKLLIYYTSRARSGVPSRFSGSGSGTDFTFTISSLQPEDIATYFCQQGDTLPYTFGQGTKLEIK

SEQ ID NO: 216 - protein, 107 aa, synthetic construct
  REGION 1..107: note = VL Domain oif of hCD137 MAB-3 VL9
DIQMTQSPSSLSASVGDRVTITCQASQDISNYLNWYQQKPDKTVKLLIYYTSRARSGVPSRFSGSGSGTDFTFTISSLQPEDIATYFCQQGDTLPYTFGQGTKLEIK

SEQ ID NO: 217 - protein, 107 aa, synthetic construct
  REGION 1..107: note = VL Domain oif of hCD137 MAB-3 VL10
DIQMTQSPSSLSASVGDRVTITCRPSQDISNYLNWYQQKPDKTVKLLIYYTTRLRSGVPSRFSGSGSGTDFTFTISSLQPEDIATYFCQQGDTLPYTFGQGTKLEIK

SEQ ID NO: 218 - protein, 107 aa, synthetic construct
  REGION 1..107: note = VL Domain oif of hCD137 MAB-3 VL11
DIQMTQSPSSLSASVGDRVTITCRPSQDISNYLNWYQQKPDKTVKLLIYYTGRLRSGVPSRFSGSGSGTDFTFTISSLQPEDIATYFCQQGDTLPYTFGQGTKLEIK

SEQ ID NO: 219 - protein, 107 aa, synthetic construct
  REGION 1..107: note = VL Domain oif of hCD137 MAB-3 VL12
DIQMTQSPSSLSASVGDRVTITCRPSQDISNYLNWYQQKPDKTVKLLAYYTTRLRSGVPSRFSGSGSGTDFTFTISSLQPEDIATYFCQQGDTLPYTFGQGTKLEIK

SEQ ID NO: 220 - protein, 107 aa, synthetic construct
  REGION 1..107: note = VL Domain oif of hCD137 MAB-3 VL13
DIQMTQSPSSLSASVGDRVTITCRPSQDISNYLNWYQQKPDKTVKLLAYYTGRLRSGVPSRFSGSGSGTDFTFTISSLQPEDIATYFCQQGDTLPYTFGQGTKLEIK

SEQ ID NO: 221 - protein, 107 aa, synthetic construct
  REGION 1..107: note = VL Domain oif of hCD137 MAB-3 VL14
DIQMTQSPSSLSASVGDRVTITCQASQDISNYLNWYQQKPDKTVKLLIYYTTRARSGVPSRFSGSGSGTDFTFTISSLQPEDIATYFCQQGDTLPYTFGQGTKLEIK

SEQ ID NO: 222 - protein, 107 aa, synthetic construct
  REGION 1..107: note = VL Domain oif of hCD137 MAB-3 VL15
DIQMTQSPSSLSASVGDRVTITCQASQDISNYLNWYQQKPDKTVKLLIYYTGRARSGVPSRFSGSGSGTDFTFTISSLQPEDIATYFCQQGDTLPYTFGQGTKLEIK

SEQ ID NO: 223 - protein, 11 aa, synthetic construct
  REGION 1..11: note = CDRL1 of hCD137 MAB-3 VL4, hCD137 MAB-3 VL7, hCD137 MAB-3 VL8, hCD137 MAB-3 VL9, hCD137 MAB-3 VL14 and hCD137 MAB-3 VL15
QASQDISNYLN

SEQ ID NO: 224 - protein, 7 aa, synthetic construct
  REGION 1..7: note = CDRL2 of hCD137 MAB-3 VL6, hCD137 MAB-3 VL8 and hCD137 MAB-3 VL9
YTSRARS

SEQ ID NO: 225 - protein, 7 aa, synthetic construct
  REGION 1..7: note = CDRL2 of hCD137 MAB-3 VL10 and hCD137 MAB-3 VL12
YTTRLRS

SEQ ID NO: 226 - protein, 7 aa, synthetic construct
  REGION 1..7: note = CDRL2 of hCD137 MAB-3 VL11 and hCD137 MAB-3 VL13
YTGRLRS

SEQ ID NO: 227 - protein, 7 aa, synthetic construct
  REGION 1..7: note = CDRL2 of hCD137 MAB-3 VL14
YTTRARS

SEQ ID NO: 228 - protein, 7 aa, synthetic construct
  REGION 1..7: note = CDRL2 of hCD137 MAB-3 VL15
YTGRARS

SEQ ID NO: 229 - protein, 497 aa, synthetic construct
  REGION 1..497: note = First Polypeptide Chain of TRIDENT-A5
DIQMTQSPSSLSASVGDRVTITCQASQDISNYLNWYQQKPDKTVKLLIYYTGRARSGVPSRFSGSGSGTDFTFTISSLQPEDIATYFCQQGDTLPYTFGQGTKLEIKGGGSGGGGQVQLVQSGAEVKKPGASVKVSCKASGYTFTSYWINWVRQAPGQGLEWIGNIYPSDSYTNYNQKFKDKATITADKSTSTAYMELSSLRSEDTAVYYCTRDYGSAYSMSTWGQGTTVTVSSASTKGEVAACEKEVAALEKEVAALEKEVAALEKGGGDKTHTCPPCPAPEAAGGPSVFLFPPKPKDTLMISRTPEVTCVVVDVSHEDPEVKFNWYVDGVEVHNAKTKPREEQYNSTYRVVSVLTVLHQDWLNGKEYKCKVSNKALPAPIEKTISKAKGQPREPQVYTLPPSREEMTKNQVSLWCLVKGFYPSDIAVEWESNGQPENNYKTTPPVLDSDGSFFLYSKLTVDKSRWQQGNVFSCSVMHEALHNHYTQKSLSLSPGK

SEQ ID NO: 230 - protein, 267 aa, synthetic construct
  REGION 1..267: note = Second Polypeptide Chain of TRIDENT-A5
DIQMTQSPSSLSASVGDRVTITCQASQDISNYLNWYQQKPDKTVKLLIYYTGRARSGVPSRFSGSGSGTDFTFTISSLQPEDIATYFCQQGDTLPYTFGQGTKLEIKGGGSGGGGQVQLVQSGAEVKKPGASVKVSCKASGYTFTSYWINWVRQAPGQGLEWIGNIYPSDSYTNYNQKFKDKATITADKSTSTAYMELSSLRSEDTAVYYCTRDYGSAYSMSTWGQGTTVTVSSASTKGKVAACKEKVAALKEKVAALKEKVAALKE

SEQ ID NO: 231 - protein, 448 aa, synthetic construct
  REGION 1..448: note = Third Polypeptide Chain of TRIDENT-B
QVQLVQSGAEVKKPGASVKVSCKASGYTFTSFWMHWVRQAPGQGLEWMGRIDPNRGGTEYNEKAKSRVTMTADKSTSTAYMELSSLRSEDTAVYYCAGGNPYYPMDYWGQGTTVTVSSASTKGPSVFPLAPSSKSTSGGTAALGCLVKDYFPEPVTVSWNSGALTSGVHTFPAVLQSSGLYSLSSVVTVPSSSLGTQTYICNVNHKPSNTKVDKRVEPKSCDKTHTCPPCPAPEAAGGPSVFLFPPKPKDTLMISRTPEVTCVVVDVSHEDPEVKFNWYVDGVEVHNAKTKPREEQYNSTYRVVSVLTVLHQDWLNGKEYKCKVSNKALPAPIEKTISKAKGQPREPQVYTLPPSREEMTKNQVSLSCAVKGFYPSDIAVEWESNGQPENNYKTTPPVLDSDGSFFLVSKLTVDKSRWQQGNVFSCSVMHEALHNRYTQKSLSLSPGK

SEQ ID NO: 232 - protein, 214 aa, synthetic construct
  REGION 1..214: note = Fourth Polypeptide Chain of TRIDENT-B
DIQMTQSPSSLSASVGDRVTITCRASQGISNYLAWFQQKPGKAPKSLIYRANRLQSGVPSRFSGSGSGTDFTLTISSLQPEDVATYYCLQYDDFPWTFGQGTKLEIKRTVAAPSVFIFPPSDEQLKSGTASVVCLLNNFYPREAKVQWKVDNALQSGNSQESVTEQDSKDSTYSLSSTLTLSKADYEKHKVYACEVTHQGLSSPVTKSFNRGEC